European Patent Application EP 4 759 928 A1, published June 17, 2026. Title: 瓦伦烯合成酶及其应用. Applicant: 武汉合生科技有限公司. Application CN. The sequence listing filed with the application follows.

SEQUENCE LISTING (178 sequences)

SEQ ID NO: 1 - protein, 555 aa, Actaea racemosa
MEVTRRSANYHPSVWGDKFLEYSSPDHLKNDSDHLKNDAVTEKKHEKLKEEVKKMLVETVQKPQQQLNLINEIQRLGLSFHFEPEIEAALRQISVTYHEYCCSTNVDDLHNVALCFRILREHGHKVSCDVFHKFMDSNGKLKGSFLNDAIGLLSLYEATHFRVHGEDLLEDVLSLTTSRLEYLKSQMKYPLEDEITRALKHPLHKELNRLGARYYISIYEKYDSHNKLLLEFAKLDFNRMQKMYQHELAELTRWWKDLDFTNKLPFARDRIVEGYFWILGMYFEPECKDVREFLNRVFALISVVDDTYDVYGTFEEVILFTHAIERWETSALDQLPEYMKIIYQALMDVYSQMEEKLAKKADCPTYRLEFAIETVKALFRSYLEEARWSKERYIPTMEEYMTVALVSVGYKTILTNSFVGMGDTATREVFEWVFSSPLIVRASDLIARLGDDIGGHEEEQKKGDAATAVECYMKEHGVTKQEAYAEFQKQIDNAWKDLNQEALRPFPVPMTYITRVVHFTRAIHVIYADSDDGYTRPEKKIKGYITSLLVDPIPM

SEQ ID NO: 2 - protein, 572 aa, Actaea racemosa
MSLNVLSTSGSAPTTKSSEVTRRSANYHPSVWGDKFLEYSSPDHLKNDSDHLKNDAVTEKKHEKLKEEVKKMLVETVQKPQQQLNLINEIQRLGLSFHFEPEIEAALRQISVTYHEYCCSTNVDDLHNVALCFRILREHGHKVSCDVFHKFMDSNGKLKGSFLNDAIGLLSLYEATHFRVHGEDLLEDVLSLTTSRLEYLKSQMKYPLEDEITRALKHPLHKELNRLGARYYISIYEKYDSHNKLLLEFAKLDFNRMQKMYQHELAELTRWWKDLDFTNKLPFARDRIVEGYFWILGMYFEPECKDVREFLNRVFALISVVDDTYDVYGTFEEVILFTHAIERWETSALDQLPEYMKIIYQALMDVYSQMEEKLAKKADCPTYRLEFAIETVKALFRSYLEEARWSKERYIPTMEEYMTVALVSVGYKTILTNSFVGMGDTATREVFEWVFSSPLIVRASDLIARLGDDIGGHEEEQKKGDAATAVECYMKEHGVTKQEAYAEFQKQIDNAWKDLNQEALRPFPVPMTYITRVVHFTRAIHVIYADSDDGYTRPEKKIKGYITSLLVDPIPM

SEQ ID NO: 3 - protein, 548 aa, Citrus maxima
MSSGETFRPTADFHPSLWRNHFLKGASDFKTVDHTATQERHEALKEEVRRMITDAEDKPVQKLRLIDEVQRLGVAYHFEKEIEDAIQKLCPNYIHSNSPDLHTVSLHFRLLRQQGIKISCDVFEKFKDDEGRFKSSLINDVQGMLSLYEAAYMAVRGEHILDEAIAFTTTHLKSLVAQDHVTPKLAEQINHALYRPLRKTLPRLEARYFMSMINSTSDHLYNKTLLNFAKLDFNILLELHKEELNELTKWWKELDFTTKLPYARDRLVELYFWDLGTYFEPQYAFGRKIMTQLNYILSIIDDTYDAYGTLEELSLFTEAVQRWNIEAVDTLPEYMKLIYRTLLDAFNEIEEDMAKQGRSHCVRYAKEANQKVIGAYFVQAKWFSEGYVPTIEEYMPIALTSCAYTFVITNSFLGMGDFATKEVFEWISDNPKVVKAASVICRLLDDMQGHEFEQKRGHVASAIECYTKQHGVSKEEAIKMFEEEVANAWKDINEELMMKPTVVARPLLGTILNLARAIDFIYKEDDGYTHSYLIKDQIASVLGDHVPF

SEQ ID NO: 4 - DNA, 1668 bp, synthetic construct
  source 1..1668: mol_type = other DNA
atggaagttaccagaagaagtgccaactaccacccatctgtctggggtgacaagttcttggaatactcttctccagaccatttgaagaacgactccgatcacttgaagaacgacgctgtcactgaaaagaagcacgaaaagttgaaggaagaagtcaaaaagatgttggtcgaaactgtccaaaagccacaacaacaattgaacttaatcaacgaaatccaaagattgggtttgtccttccacttcgaaccagaaatcgaagctgccttaagacaaatctccgtcacatatcacgaatactgttgttctaccaacgttgatgacttgcacaacgtcgctttgtgtttcagaatcttgagagaacacggtcacaaggtttcctgcgatgtcttccataagttcatggactctaacggtaagttgaaaggttctttcttgaacgacgctatcggtttattgagcttgtacgaagctactcacttccgtgttcacggtgaagatttgttggaagatgtattatccttgactacctctagattggaataccttaagtctcagatgaagtacccattagaagacgaaataaccagagctctcaagcatccactccacaaggaattgaacagattgggtgctagatactacatttccatttacgaaaaatacgattcccacaacaagttattgctggaatttgctaagttggatttcaacagaatgcaaaaaatgtaccaacacgaattggctgagttgactagatggtggaaggaccttgacttcactaataagctacctttcgccagagacagaatcgttgaaggttacttctggattttgggtatgtactttgaaccagaatgtaaggacgttagagaatttttgaacagagtttttgctttaatctctgttgtcgatgatacatacgacgtctacggtactttcgaagaagttattttattcacccacgctattgaacgttgggaaacttccgccttggaccaattgccagaatatatgaagatcatttaccaagctttgatggatgtttactcccaaatggaagaaaagttggccaagaaggctgactgtccaacctacagattggaatttgccattgaaaccgttaaggctttgttcagatcttacttggaagaagcccgttggtcaaaggaaagatatattccaaccatggaggaatatatgactgttgctttggtttctgttggttacaagactatcttgactaactctttcgttggtatgggtgacactgctaccagagaagttttcgaatgggttttctcctccccattgattgtcagagcttctgatttgattgctaggttgggcgacgacattggtggtcacgaagaagaacaaaagaagggtgatgccgctaccgctgtcgaatgttacatgaaagaacatggtgtcaccaagcaagaagcttacgccgaattccaaaagcaaattgacaacgcttggaaggacttaaaccaagaagccttaagaccattcccagttccaatgacctacatcactcgtgttgttcatttcaccagagctattcacgttatctacgctgatagtgacgatggttacacccgtcctgaaaagaaaatcaagggttacatcacttctttgttggtagacccaatcccaatgtga

SEQ ID NO: 5 - DNA, 1719 bp, synthetic construct
  source 1..1719: mol_type = other DNA
atgtcgttaaatgtgctatccacttctggttctgctccaactaccaaatcttctgaagttaccagaagaagtgccaactaccacccatctgtctggggtgacaagttcttggaatactcttctccagaccatttgaagaacgactccgatcacttgaagaacgacgctgtcactgaaaagaagcacgaaaagttgaaggaagaagtcaaaaagatgttggtcgaaactgtccaaaagccacaacaacaattgaacttaatcaacgaaatccaaagattgggtttgtccttccacttcgaaccagaaatcgaagctgccttaagacaaatctccgtcacatatcacgaatactgttgttctaccaacgttgatgacttgcacaacgtcgctttgtgtttcagaatcttgagagaacacggtcacaaggtttcctgcgatgtcttccataagttcatggactctaacggtaagttgaaaggttctttcttgaacgacgctatcggtttattgagcttgtacgaagctactcacttccgtgttcacggtgaagatttgttggaagatgtattatccttgactacctctagattggaataccttaagtctcagatgaagtacccattagaagacgaaataaccagagctctcaagcatccactccacaaggaattgaacagattgggtgctagatactacatttccatttacgaaaaatacgattcccacaacaagttattgctggaatttgctaagttggatttcaacagaatgcaaaaaatgtaccaacacgaattggctgagttgactagatggtggaaggaccttgacttcactaataagctacctttcgccagagacagaatcgttgaaggttacttctggattttgggtatgtactttgaaccagaatgtaaggacgttagagaatttttgaacagagtttttgctttaatctctgttgtcgatgatacatacgacgtctacggtactttcgaagaagttattttattcacccacgctattgaacgttgggaaacttccgccttggaccaattgccagaatatatgaagatcatttaccaagctttgatggatgtttactcccaaatggaagaaaagttggccaagaaggctgactgtccaacctacagattggaatttgccattgaaaccgttaaggctttgttcagatcttacttggaagaagcccgttggtcaaaggaaagatatattccaaccatggaggaatatatgactgttgctttggtttctgttggttacaagactatcttgactaactctttcgttggtatgggtgacactgctaccagagaagttttcgaatgggttttctcctccccattgattgtcagagcttctgatttgattgctaggttgggcgacgacattggtggtcacgaagaagaacaaaagaagggtgatgccgctaccgctgtcgaatgttacatgaaagaacatggtgtcaccaagcaagaagcttacgccgaattccaaaagcaaattgacaacgcttggaaggacttaaaccaagaagccttaagaccattcccagttccaatgacctacatcactcgtgttgttcatttcaccagagctattcacgttatctacgctgatagtgacgatggttacacccgtcctgaaaagaaaatcaagggttacatcacttctttgttggtagacccaatcccaatgtga

SEQ ID NO: 6 - DNA, 1647 bp, synthetic construct
  source 1..1647: mol_type = other DNA
atgtcttctggtgaaactttcagaccaactgctgatttccacccatctttgtggagaaaccacttcttgaagggtgccagcgacttcaaaactgttgaccacactgccacccaagaaagacacgaagctttgaaagaagaagtcagacgtatgattactgacgctgaagacaagccagttcaaaagctaagattgatagacgaagtccaaagattaggtgttgcttaccattttgaaaaggaaatcgaagatgctatccaaaagttatgtccaaactacattcactccaactctccagacttgcacactgtcagtcttcatttcaggttgttgagacaacaaggtatcaagatctcttgtgatgtcttcgaaaagttcaaggatgacgaaggtagattcaagtcctcactgattaacgatgttcaaggtatgttgtccttgtacgaagccgcctacatggctgttagaggtgaacacattttggatgaagccatcgctttcaccaccactcacttgaagtctctagtggctcaggatcatgttaccccaaagttggctgaacaaatcaatcacgctctctaccgtcctttaagaaagactttgccaagattggaagctcgttacttcatgtccatgatcaactccacttctgaccatttgtacaacaagactctattgaacttcgctaaattggacttcaacatattgttggaattgcacaaggaagaattgaatgaactgactaaatggtggaaggaattagattttactacaaagttgccatacgctagagacagattggttgaattatatttctgggacttaggcacatacttcgaaccacaatacgccttcggtagaaagattatgactcaattgaactacatcttgagcatcattgacgacacttacgacgcttacggtactttagaagagttgtccttgttcactgaagccgtccaaagatggaacattgaagcagtcgataccttgccagaatatatgaaattgatctacagaaccttgttagatgcttttaacgaaattgaagaagacatggccaaacaaggtcgttcccattgtgtcagatacgctaaggaagctaaccaaaaggtcattggtgcttacttcgttcaagctaagtggttctctgaaggttacgttccaaccattgaagaatatatgccaatcgccctcacctcttgcgcttacacttttgtcatcaccaactctttcttgggtatgggtgactttgctaccaaggaagtctttgaatggatttctgacaacccaaaggttgtcaaggctgcttctgttatctgtagattgttggatgatatgcaaggtcacgaattcgagcaaaagagaggtcacgttgcttctgctatcgaatgttacaccaagcaacacggtgtctccaaggaagaagctatcaagatgttcgaagaagaagttgccaacgcttggaaggacattaacgaagaactgatgatgaagcctaccgttgttgctagaccattgttgggtaccatcttgaacttggccagagctattgatttcatctacaaggaagatgatggttacacccactcttacttgattaaggaccaaattgcttccgttttgggtgaccacgtcccattctga

SEQ ID NO: 7 - DNA, 58 bp, synthetic construct
  source 1..58: mol_type = other DNA
ctaattacatgatatcgacaaaggaaaaggggcctgttcacattgggattgggtctac

SEQ ID NO: 8 - DNA, 51 bp, synthetic construct
  source 1..51: mol_type = other DNA
gtaagaatttttgaaaattcaatataaatggaagttaccagaagaagtgcc

SEQ ID NO: 9 - DNA, 58 bp, synthetic construct; identical to SEQ ID NO: 7
  source 1..58: mol_type = other DNA

SEQ ID NO: 10 - DNA, 53 bp, synthetic construct
  source 1..53: mol_type = other DNA
gtaagaatttttgaaaattcaatataaatgtcgttaaatgtgctatccacttc

SEQ ID NO: 11 - DNA, 50 bp, synthetic construct
  source 1..50: mol_type = other DNA
catgatatcgacaaaggaaaaggggcctgttcagaatgggacgtggtcac

SEQ ID NO: 12 - DNA, 53 bp, synthetic construct
  source 1..53: mol_type = other DNA
agtaagaatttttgaaaattcaatataaatgtcttctggtgaaactttcagac

SEQ ID NO: 13 - DNA, 46 bp, synthetic construct
  source 1..46: mol_type = other DNA
cgacaaaggaaaaggggcctgttcaaatgacagcgttgatgaaaac

SEQ ID NO: 14 - DNA, 50 bp, synthetic construct
  source 1..50: mol_type = other DNA
gtaagaatttttgaaaattcaatataaatgtccactcaagtttcagccag

SEQ ID NO: 15 - DNA, 45 bp, synthetic construct
  source 1..45: mol_type = other DNA
tatcgacaaaggaaaaggggcctgttcagaatgggacgtggtcac

SEQ ID NO: 16 - DNA, 46 bp, synthetic construct
  source 1..46: mol_type = other DNA
aagaatttttgaaaattcaatataaatgtcttctggtgaaaccttc

SEQ ID NO: 17 - DNA, 52 bp, synthetic construct
  source 1..52: mol_type = other DNA
tatcgacaaaggaaaaggggcctgttcagataattgggtcaactaaaatatc

SEQ ID NO: 18 - DNA, 49 bp, synthetic construct
  source 1..49: mol_type = other DNA
aagaatttttgaaaattcaatataaatggaattatgcactcaaaccgtc

SEQ ID NO: 19 - DNA, 45 bp, synthetic construct
  source 1..45: mol_type = other DNA
acaaaggaaaaggggcctgttcaaatgataggatcgacaagaatg

SEQ ID NO: 20 - DNA, 45 bp, synthetic construct
  source 1..45: mol_type = other DNA
tttttgaaaattcaatataaatggaattgtgtactcaaactgttg

SEQ ID NO: 21 - DNA, 45 bp, synthetic construct
  source 1..45: mol_type = other DNA
acaaaggaaaaggggcctgttcagatggctggaccatttagaaac

SEQ ID NO: 22 - DNA, 43 bp, synthetic construct
  source 1..43: mol_type = other DNA
tttttgaaaattcaatataaatggccgcctccgaagccgcctc

SEQ ID NO: 23 - DNA, 59 bp, synthetic construct
  source 1..59: mol_type = other DNA
catgatatcgacaaaggaaaaggggcctgtttaaggaataataggttcaacaaagaact

SEQ ID NO: 24 - DNA, 59 bp, synthetic construct
  source 1..59: mol_type = other DNA
tccaaaaaaaaagtaagaatttttgaaaattcaatataaatggctgaaatgttcaacgg

SEQ ID NO: 25 - DNA, 59 bp, synthetic construct
  source 1..59: mol_type = other DNA
tacatgatatcgacaaaggaaaaggggcctgtttataatggaattggatcaaccaacaa

SEQ ID NO: 26 - DNA, 59 bp, synthetic construct
  source 1..59: mol_type = other DNA
aaaagtaagaatttttgaaaattcaatataaatgtcattgaatgttttatctacatcag

SEQ ID NO: 27 - DNA, 48 bp, synthetic construct
  source 1..48: mol_type = other DNA
acaaaggaaaaggggcctgtttaaattgggatagattcaaccaaaacc

SEQ ID NO: 28 - DNA, 46 bp, synthetic construct
  source 1..46: mol_type = other DNA
aatttttgaaaattcaatataaatggaaaagcaatctgttacattg

SEQ ID NO: 29 - protein, 556 aa, Vitis vinifera
MSTQVSASSLAQIPQPKNRPVANFHPNIWGDQFITYTPEDKVTRACKEEQIEDLKKEVKRKLTAAAVANPSQLLNFIDAVQRLGVAYHFEQEIEEALQHICNSFHDCNDMDGDLYNIALGFRLLRQQGYTISCDIFNKFTDERGRFKEALISDVRGMLGLYEAAHLRVHGEDILAKALAFTTTHLKAMVESLGYHLAEQVAHALNRPIRKGLERLEARWYISVYQDEAFHDKTLLELAKLDFNLVQSLHKEELSNLARWWKELDFATKLPFARDRLVEGYFWMHGVYFEPQYLRGRRILTKVIAMTSILDDIHDAYGTPEELKLFIEAIERWDINSINQLPEYMKLCYVALLDVYKEIEEEMEKEGNQYRVHYAKEVMKNQVRAYFAEAKWLHEEHVPAFEEYMRVALASSGYCLLATTSFVGMGEIATKEAFDWVTSDPKIMSSSNFITRLMDDIKSHKFEQKRGHVASAVECYMKQYGVSEEQVYSEFQKQIENAWLDINQECLKPTAVSMPLLARLLNLTRTMDVIYKEQDSYTHVGKVMRDNIASVFINAVI

SEQ ID NO: 30 - DNA, 1671 bp, synthetic construct
  source 1..1671: mol_type = other DNA
atgtccactcaagtttcagccagctccttagctcaaattccacaaccaaagaacagacctgttgctaacttccatccaaacatctggggtgaccaattcatcacttacactccagaagacaaggttactcgtgcttgtaaggaagaacaaattgaagatttgaagaaggaagtcaagagaaagttgactgctgctgccgtcgccaacccatctcaattattgaactttattgacgctgtccaaagattgggtgtcgcctaccacttcgaacaagaaattgaagaagcattgcaacacatctgtaattcttttcatgactgtaacgacatggacggtgacttgtacaacattgctctcggtttcagacttttaagacaacaaggttacaccatttcttgtgatatcttcaataaattcactgatgaacgtggtagattcaaggaggctttgatctctgacgttagaggtatgttgggtttgtacgaagctgctcatttgagagtccacggtgaagatatactggccaaggctttggcgtttaccaccactcacttgaaggctatggttgaatctttgggctaccacttggctgaacaagttgctcacgctttgaacagaccaatcagaaagggtttggaaagattggaagccagatggtacatctctgtctaccaagacgaagctttccacgacaagactttgttggaattggctaagttggatttcaacttggttcaatccttgcataaagaagaattgtccaatttagccagatggtggaaggagctggattttgctaccaagttgccattcgctcgtgacagattagtcgaaggttacttctggatgcacggtgtttacttcgaaccacaatacttgagaggtagaagaattttgacaaaggtcatcgctatgacttctatcttggatgacattcacgatgcttacggtactcctgaagaactaaaattattcattgaagccattgaaagatgggatattaactccatcaaccagttgccagaatatatgaaattgtgttacgttgctttgttggatgtatacaaggaaatcgaagaagaaatggaaaaggaaggtaaccaatacagagttcactacgctaaggaagtaatgaagaaccaagtcagagcttatttcgctgaagctaagtggttgcacgaagaacacgttccagcttttgaagaatacatgagagttgctttggcttcctctggttactgtttgcttgctactacctctttcgttggtatgggtgaaattgccaccaaggaagccttcgactgggtcacctctgacccaaagatcatgtcttcttctaacttcatcaccagattgatggatgatatcaagtctcacaagttcgaacaaaagcgtggtcacgttgcctcagctgttgagtgctacatgaagcaatatggtgtttccgaagaacaagtctactctgaattccaaaaacaaatcgaaaacgcttggttagacattaaccaagaatgtttgaagccaaccgctgtctccatgccattgttggctcgtctattaaacttgaccagaaccatggacgttatctacaaagaacaagattcttacactcacgttggtaaggtcatgagagacaacatcgcctccgttttcatcaacgctgtcatttga

SEQ ID NO: 31 - protein, 548 aa, Citrus sinensis
MSSGETFRPTADFHPSLWRNHFLKGASDFKTVDHTATQERHEALKEEVRRMITDAEDKPVQKLRLIDEVQRLGVAYHFEKEIGDAIQKLCPIYIDSNRADLHTVSLHFRLLRQQGIKISCDVFEKFKDDEGRFKSSLINDVQGMLSLYEAAYMAVRGEHILDEAIAFTTTHLKSLVAQDHVTPKLAEQINHALYRPLRKTLPRLEARYFMSMINSTSDHLCNKTLLNFAKLDFNILLELHKEELNELTKWWKDLDFTTKLPYARDRLVELYFWDLGTYFEPQYAFGRKIMTQLNYILSIIDDTYDAYGTLEELSLFTEAVQRWNIEAVDMLPEYMKLIYRTLLDAFNEIEEDMAKQGRSHCVRYAKEENQKVIGAYSVQAKWFSEGYVPTIEEYMPIALTSCAYTFVITNSFLGMGDFATKEVFEWISNNPKVVKAASVICRLMDDMQGHEFEQKRGHVASAIECYTKQHGVSKEEAIKMFEEEVANAWKDINEELMMKPTVVARPLLGTILNLARAIDFIYKEDDGYTHSYLIKDQIASVLGDHVPF

SEQ ID NO: 32 - DNA, 1647 bp, synthetic construct
  source 1..1647: mol_type = other DNA
atgtcttctggtgaaaccttcaggccaactgccgacttccacccatccttgtggagaaaccattttttgaagggtgcctctgatttcaagactgtcgaccacactgctacccaagaaagacacgaagctttgaaggaagaagtcagaagaatgatcactgacgctgaggacaagccagtccaaaagttgcgtctgattgacgaagttcaaagattgggtgtcgcttaccacttcgaaaaggaaattggtgatgctattcaaaaactatgtccaatctacattgactccaacagagctgacttgcacaccgtttccttacacttcagattattgagacaacaaggtatcaagatttcttgtgatgttttcgaaaagttcaaggatgatgaaggtagattcaagtctagtttgattaacgatgtccaaggtatgttgtccttgtacgaagccgcttacatggctgttagaggtgaacacattttggatgaagctatcgcttttaccacaacccacttgaagtcccttgttgctcaagatcatgttactccaaagttagccgaacaaatcaaccacgctttatacagaccattgagaaagaccctaccaagattggaagccagatacttcatgtccatgattaatagcacttccgaccatttgtgtaacaagaccttactgaactttgctaaattggacttcaacatcttattggaattgcacaaggaagaattaaacgaattgactaagtggtggaaggatttggacttcacaactaagttgccatacgctagagacagattggttgaattgtatttctgggatttgggtacttacttcgaaccacaatacgccttcggtagaaagatcatgactcaattgaactacatcttgtctatcattgatgacacctacgatgcctacggtactttggaagaactatcattattcactgaagctgttcaaagatggaacatcgaagctgtcgatatgttaccagaatatatgaaattgatttacagaaccttgttggatgctttcaacgaaatcgaagaagacatggccaaacaaggacgttctcattgtgttcgttatgctaaagaagaaaaccaaaaggtcattggtgcttactctgtccaagctaaatggttctctgaaggttacgttcctaccatcgaagaatacatgccaattgctttgacttcctgcgcttacactttcgttatcaccaactctttcttgggtatgggtgattttgctactaaggaagtctttgaatggatctctaacaacccaaaggttgttaaggctgcttccgttatctgtagattgatggacgacatgcaaggtcacgaattcgaacaaaagagaggtcatgttgcttctgctattgaatgttacaccaagcaacacggtgtttctaaggaagaagctatcaagatgttcgaagaggaagtcgccaacgcttggaaggacatcaatgaagaattgatgatgaaacctaccgtcgtagcccgtccattgttgggcaccattttgaacttggctagagctattgacttcatctacaaggaagatgacggttacactcactcttacttaatcaaggaccaaattgcgtccgttttgggtgaccacgtcccattctga

SEQ ID NO: 33 - protein, 554 aa, Solanum habrochaites
MELCTQTVAADHEVIITRRSGSHHPTLWGDHFLAYADLRGANEGEEKQNEDLKEEVRKMLVMAPSNSLEKLELINTIQCLGLAYHFQSEIDESLSYMYTHYEEYSIGDLHAIALCFRLLRQQGYYVSCDAFKKFTNDQGNFKEELVKDVEGMLSLYEAAQFRVHGEQILDEALNFTITKLKQILPKLSNSQLAQQITNALKFPIKDGIVRVETRKYISFYQQNQNHNQVLLNFAKLDFNILQTLHKKELSDMTRWWKKMELVNTLPYARDRLVECYFWCLGTYFEPQYSVARKMLTKISFFISIIDDTYDIYGKLDELTLFTQAIERWNIDASEQLPLYMKIIYRDLLDVYDEIEKELANENKSFLVNYSINEMKKVVRGYFQEAKWYYGKKVPKMEQYMKNAISTSAYILLTTTSWLAMGNVATKDVFDWVATEPKLVVASCHIIRLLNDLVSHEEEQKRGNAASAVECYMNEYSVTQEEAHVKIRDIIENYWKDLNEEYFKVDMIIIPRVLLMCIINLTRVAEFIYKDEDAYTFSKNNLKDVISDILVDPII

SEQ ID NO: 34 - DNA, 1665 bp, synthetic construct
  source 1..1665: mol_type = other DNA
atggaattatgcactcaaaccgtcgctgccgaccacgaagttatcattaccagaagatctggttcccatcatccaactttgtggggtgaccatttcctggcttacgccgatttgagaggtgctaacgaaggtgaagaaaagcaaaacgaagatttgaaggaagaagtcagaaagatgttggttatggctccatctaactctttggaaaagttggaattgatcaacactatccaatgtttgggcttggcttaccacttccaatctgaaatcgacgaatccttgagctacatgtacactcactacgaggaatactctattggtgaccttcacgctatcgctttgtgtttccgtttgttgagacaacaaggttactacgtttcttgtgatgctttcaaaaaattcaccaacgaccaaggtaacttcaaggaagaattggttaaggatgttgaaggtatgttgtctttgtacgaagctgcccaattcagagttcacggtgaacaaattttggacgaagctttgaatttcactattacaaagttgaagcaaatcttgccaaagttgtccaactctcaattagctcaacaaatcactaacgccctaaagttcccaatcaaggacggtattgtccgtgttgaaaccagaaagtacatctcattctaccaacagaaccaaaaccacaaccaagttttattgaactttgctaagttggatttcaacattttgcaaactttacacaagaaggagttgtctgacatgactagatggtggaaaaagatggaactcgttaatacgttgccatacgctagagacagattggttgaatgttacttctggtgtttgggtacttacttcgaaccacaatactccgttgctcgtaaaatgctgaccaagatttctttcttcatctctatcattgatgacacctacgacatttacggtaagttggatgaattgaccttgtttactcaagctattgaaagatggaacattgatgcttccgaacaattgcctttatacatgaaaatcatctacagagacttgttagatgtctacgatgaaattgaaaaggaattggctaacgaaaacaagtcctttttggtcaattactctatcaacgaaatgaagaaggtcgttcgtggttactttcaagaagccaagtggtactatggtaagaaggtaccaaagatggaacaatatatgaagaacgccattagtacttccgcctacattcttttgaccactacttcttggttagctatgggtaacgttgccaccaaggacgtcttcgactgggttgctactgaaccaaaattggttgtcgcctcctgtcacatcattagattgttgaacgatttagtctctcacgaagaagaacaaaagagaggtaacgccgcttctgctgtcgaatgttacatgaacgaatactccgttacccaagaagaagctcacgtcaagatcagagatatcatcgaaaactactggaaggacctgaatgaggaatatttcaaggtcgatatgattattattccaagagtcttgttgatgtgtatcatcaacttgaccagagttgctgaattcatctacaaggacgaagacgcttacaccttctctaagaacaacctaaaagacgtcatctcagatattttagttgacccaattatctga

SEQ ID NO: 35 - protein, 554 aa, Solanum lycopersicum
MELCTQTVAADHEVIITRRSGSHHPTLWGDHFLAYADLRGANEGEEKQNEDLKEEVRKMLVMAPSKSLEKLELINTIQCLGLGYHFQSEIDESLSYMYTHYEEYSIGDLHAIALCFRLLRQQGYYVSCDAFKKFTNDQGNFKEELVKDVEGMLSLYEAAQFRVHGEQILDEALNFTIAQLKQILPKLSNSQLAQQITNALKYPIKDGIVRVETRKYISFYQQNQNHNEVLLNFAKLDFNILQTLHKKELSDMTRWWKKMELVNTLPYARDRLVECYFWCLGTYFEPQYSVARKMLTKISFYISIIDDTYDIYGKLDELTLFTQAIERWNIDASEQLPLYMKIIYRDLLDVYDEIEKELANENKSFLVNYSINEMKKVVRGYFQEAKWYYGKKVPTMEQYMKNGISTSAYILLTTTSWLAMGNVATKDAFDWVATEPPIVVASCYIIRLLNDLVSHEEEQKRGNAASAVECYMNEYSVTKEEAHIKIRDIIENYWKDLNEEYFKVDMIIIPRVLLMCIINLTRVAEFIYKDEDAYTFSKNNLKDVISDILVDPII

SEQ ID NO: 36 - DNA, 1665 bp, synthetic construct
  source 1..1665: mol_type = other DNA
atggaattgtgtactcaaactgttgctgctgatcacgaagttataatcaccagaagatctggctctcatcacccaactttgtggggtgaccatttcttggcttacgctgacctccgtggtgctaacgaaggtgaagaaaagcaaaacgaggatcttaaagaagaagtcagaaagatgttggttatggctccatccaagtccctcgaaaaattggaattgattaacaccatccaatgtttgggtttgggttaccacttccaatctgaaatcgacgaatctttgtcttacatgtacactcattacgaagaatactccattggtgacttgcacgctattgctctatgtttcagattgttgagacaacaaggttactacgttagctgcgatgctttcaagaagttcaccaacgaccaaggtaacttcaaggaagaattggtcaaggacgttgaaggtatgttatctttgtacgaagctgctcaattcagagtccacggtgaacaaattttggacgaagctttgaacttcactatcgctcaattgaaacaaattttgccaaagttgtccaactctcaattggcccaacaaatcactaacgccttgaagtacccaatcaaggatggtattgtccgtgtggaaaccagaaagtacatttctttctaccaacaaaaccaaaatcacaacgaagtcctgttgaactttgctaagttagacttcaacatcttgcaaaccttgcacaagaaagaattgtccgacatgactagatggtggaagaagatggaattggtcaacactttgccatacgcgagagacagattagttgaatgttatttctggtgtttgggtacttacttcgaaccacaatactccgtcgctagaaagatgttgaccaagatctctttctacatctcaattattgatgacacttacgatatttacggtaagttggatgaactgactttgttcacccaagctatcgaaagatggaacattgacgcaagtgaacaattaccattgtacatgaaaattatttacagagatttgttggatgtctacgacgaaattgaaaaggaattagccaatgaaaacaagtcttttttggttaactactccatcaatgaaatgaaaaaggtcgttagaggttacttccaagaagccaagtggtactatggtaagaaggttccaaccatggaacaatatatgaagaacggtatctccacttctgcctacatcttgctaaccaccacatcttggttagctatgggtaacgttgctactaaggatgcttttgactgggttgccactgaaccaccaattgttgtcgcctcttgttacatcatcagactattgaacgatttagtctcccacgaagaagaacaaaagagaggtaacgctgcctccgctgttgaatgttatatgaacgagtactctgttaccaaggaagaagctcacattaagattagagatattattgaaaattactggaaggacttgaacgaagaatacttcaaggttgacatgatcatcatcccaagagttttgttgatgtgtatcatcaacttgactcgtgtagctgaattcatctacaaggatgaagacgcttacaccttttctaagaacaacttgaaggacgttatctctgacattcttgtcgatcctatcatttga

SEQ ID NO: 37 - protein, 559 aa, Switchgrass
MAASEAASPPVSVEMMMGAAGLTGFEPCVWGDFFITLAPPFSQEAEKRMRERVEQLRGELRHRVFEAAGEAMSVADTVALVDTLERLGVDSHFREEIGAALRRVVNSGPGSCKDGDLRVVALRFRLLRQHGYWVPTDVFDRFRDDTGSFRASLSSDPGGLLSLYNAAHMATPGERVLDEAISFCRRHLESMRGELASPLAEQVSRALDIPLPRLPKRLETVRYIVEYEKEEGHDPVALELARLDFDLVRALHLEELRALSLWWKEVYGDVKLSYARDRLVENYFWTCGVFHEEEYSRARMLFAKTFGMLSLMDDTYDVYATLEECHVLNEAIQRWDESAVSTLPEYMKKFYINLLKTFQECEDSLQPDEKYRVSYAKKAFQLSSKYYLDEAKWSSEKYAPSFEEHVEVSVMSSGFPTLAVVLLMGAGDLATREAFEWAIGVPAVVSASGEVARFLNDIASYRKGKNKKDALSSVECYARERGVSGEEAAAAIAGMAEHAWRTINRSCMEVGGALLPAARLVVNLTKTLEVIYLGGRDAYTFAGDLRDLVVSLFLNGPAI

SEQ ID NO: 38 - DNA, 1680 bp, synthetic construct
  source 1..1680: mol_type = other DNA
atggccgcctccgaagccgcctccccaccagtctctgtcgaaatgatgatgggtgccgctggccttactggtttcgaaccatgcgtctggggtgatttcttcatcacattggctcctccattctctcaagaagctgaaaagagaatgagagaaagagttgaacaattgagaggtgaattgagacacagagtctttgaagccgctggtgaagctatgtccgtcgctgacactgtcgccttggtcgataccctggaaagattgggtgttgactcccacttccgtgaagaaatcggtgctgctttgagaagagttgtcaactctggtccaggttcctgtaaggatggtgacttgagagtcgttgctttgcgttttagattgctaagacaacacggttactgggttccaactgatgttttcgacagattcagagacgacaccggttctttcagagcttctttgtcttctgacccaggtggtttgctatccttgtacaacgctgctcacatggctactccaggagaacgtgttctagatgaagctatctccttctgtagacggcatttggaatccatgagaggtgaattagcttctccattggctgaacaagtttctcgtgctttggatatcccattgccaagactaccaaagagattggaaactgttagatacattgttgaatacgaaaaagaagaaggtcatgacccagttgctttggaattggctagattggacttcgatctcgtcagagctttgcacttggaggaattgagagccttatctttgtggtggaaggaagtctacggtgatgtcaagttgtcttacgctcgtgacagattggttgaaaactacttctggacttgtggtgtcttccacgaagaagaatactcaagagctagaatgttgttcgccaagaccttcggtatgttgtccttgatggacgatacttacgatgtttacgctaccctcgaagaatgtcacgttttgaacgaagctatccaaagatgggatgaatctgctgtctccactttgccagaatatatgaagaagttctacatcaacttgttgaagactttccaagaatgtgaagactctttgcaaccagacgaaaagtacagagtttcctatgccaaaaaagctttccaattatcctctaagtactacttggatgaagctaaatggtcttctgaaaagtacgctccatccttcgaagaacatgtcgaagtttccgttatgtcttctggtttcccaactttggctgttgttttgttgatgggtgctggtgacttagctaccagagaagctttcgaatgggctattggtgtacctgctgtcgtctccgcttcgggtgaagttgccagatttttgaacgatattgcttcatacagaaagggtaagaacaagaaggacgcactatcttctgttgaatgttacgccagggaaagaggcgtgtccggtgaagaagctgcagccgccattgccggtatggccgaacacgcttggagaaccattaacagaagttgtatggaagttggtggtgctcttctcccggctgctaggttggttgttaacttgaccaagaccttggaagttatttatttaggtggtcgtgatgcttacacctttgctggtgacttgagagacttagtcgtgtctttgtttctaaatggtccagccatctga

SEQ ID NO: 39 - protein, 589 aa, Callitropsis nootkatensis
MAEMFNGNSSNDGSSCMPVKDALRRTGNHHPNLWTDDFIQSLNSPYSDSSYHKHREILIDEIRDMFSNGEGDEFGVLENIWFVDVVQRLGIDRHFQEEIKTALDYIYKFWNHDSIFGDLNMVALGFRILRLNRYVASSDVFKKFKGEEGQFSGFESSDQDAKLEMMLNLYKASELDFPDEDILKEARAFASMYLKHVIKEYGDIQESKNPLLMEIEYTFKYPWRCRLPRLEAWNFIHIMRQQDCNISLANNLYKIPKIYMKKILELAILDFNILQSQHQHEMKLISTWWKNSSAIQLDFFRHRHIESYFWWASPLFEPEFSTCRINCTKLSTKMFLLDDIYDTYGTVEELKPFTTTLTRWDVSTVDNHPDYMKIAFNFSYEIYKEIASEAERKHGPFVYKYLQSCWKSYIEAYMQEAEWIASNHIPGFDEYLMNGVKSSGMRILMIHALILMDTPLSDEILEQLDIPSSKSQALLSLITRLVDDVKDFEDEQAHGEMASSIECYMKDNHGSTREDALNYLKIRIESCVQELNKELLEPSNMHGSFRNLYLNVGMRVIFFMLNDGDLFTHSNRKEIQDAITKFFVEPIIP

SEQ ID NO: 40 - DNA, 1770 bp, synthetic construct
  source 1..1770: mol_type = other DNA
atggctgaaatgttcaacggtaattcttctaatgatggttcatcatgtatgccagttaaggatgctttgaggagaactggcaatcatcaccctaacttgtggactgatgactttatacaatctttaaattctccatactcagattcttcataccataaacacagagaaattttaattgatgaaataagagatatgttttcaaacggtgagggtgatgagttcggtgttttggaaaatatatggtttgttgatgttgtccagaggttgggtattgatagacactttcaagaagagattaaaactgctttggattacatatacaaattctggaaccatgattcaattttcggtgatttgaatatggttgctttgggatttagaattttgagattaaatagatatgttgcttcttcagatgtctttaaaaaattcaaaggtgaggaaggtcaattctctggttttgaatcttctgaccaagatgcaaaattggaaatgatgttgaatttatataaggcttctgaattggattttccagatgaagatatattgaaagaagctagagcttttgcttctatgtacttgaaacatgtcattaaggaatacggtgatattcaagaatcaaagaacccattgttgatggagattgaatatacatttaagtacccttggaggtgtagattgccaagattggaggcttggaatttcattcatattatgagacaacaagattgtaacatatctttggcaaacaatttgtacaaaattcctaaaatatatatgaagaagattttggaattggctattttagatttcaatattttgcaatcacaacatcaacatgaaatgaagttgatttctacttggtggaaaaactcttctgctatacagttagatttctttcgtcatagacatattgaatcttacttctggtgggcttctcctttattcgaaccagagttttctacttgtagaattaattgtactaagttgtctactaagatgtttttgttggatgatatttacgatacttatggaactgttgaagaattgaagccatttacaacaactttaactagatgggatgtttctactgttgacaaccacccagattatatgaagattgctttcaatttttcttatgaaatttataaagaaattgcatcagaagcagagaggaagcacggtccatttgtctataaatatttgcaatcttgttggaaatcatacattgaggcttatatgcaagaagcagagtggatagcttcaaaccacattcccggttttgatgaatacttgatgaacggtgtcaaatcttctggtatgagaatattgatgattcatgctttgattttgatggatacaccattgtctgatgaaatattggaacaattagacataccatcttcaaagtcacaagccttattgtctttgattactaggttggttgatgatgttaaagatttcgaagatgaacaagctcatggtgaaatggcttcttctattgaatgttatatgaaggataaccacggttcaactagggaggacgcattgaattacttaaaaattaggattgaatcttgcgttcaagaattgaataaagaattattagagccttcaaacatgcacggttcttttcgtaatttatatttaaatgttggtatgagggttatcttttttatgttgaatgatggtgatttgtttacacattctaatagaaaagaaattcaagacgctattacaaagttctttgttgaacctattattccttaa

SEQ ID NO: 41 - protein, 565 aa, Eryngium glaciale
MSLNVLSTSGSAPTTKSSEITRRSANYHPSLWGDKFLEYSSPDHLKNDSFTEKKHEQLKEEVKKMLVETVQKPQQQLNLINEIQRLGLSYLFEPEIEAALQEISVTYDEFCCSTDADDLHNVALSFRILREHGHNVSSDVFQKFMDSNGKLKDYLVNDARGLLSLYEATHFRVHNDDKLEELLSVTTSRLEHLKSHVKYPLEDEISRALKHPLHKELNRLGARYYISIYEKFDSHNKLLLEFAKLDFNRLQKMYQHELAHLTRWWKDLDFTNKLPFARDRIVEGYFWILGMYFEPERKDVREFLNRVFALITVVDDTYDVYGTFKELLLFTDAIERWGTSDLDQLPGYMRIIYQALMDVYNQMEEKLSMKADCPTYRLEFAIETVKAMFRSYLEEARWSKEHYIPSMEEYMTVALVSVGYKTILTNSFVGMGDIATREVFEWVFNSPLIIRASDLIARLGDDIGGHEEEQKKGDAATAIECYIKENHVTKHEAYDEFQKQIDNAWKDLNKEALRPFPVPMTFITRVVHFTRAIHVIYADFSDGYTRSDKAIRGYITSLLVDPIPL

SEQ ID NO: 42 - DNA, 1698 bp, synthetic construct
  source 1..1698: mol_type = other DNA
atgtcattgaatgttttatctacatcaggttctgctccaactacaaagtcttcagaaatcactagaagatcagcaaactaccatccatctttatggggtgacaaatttttggaatactcttcaccagatcatttgaaaaatgattcttttacagaaaagaaacatgaacaattaaaagaagaagttaagaaaatgttggttgaaactgttcaaaagccacaacaacaattgaatttgattaatgaaatccaaagattgggtttgtcatacttattcgaaccagaaatcgaagctgcattgcaagaaatctcagttacttacgatgaattctgttgttctacagatgctgatgatttgcataacgttgcattgtcttttagaatcttgagagaacatggtcataatgtttcttcagatgtttttcaaaagtttatggattcaaacggtaaattgaaggattatttggttaatgatgctagaggtttgttatctttgtacgaagcaacacattttagagttcataacgatgataagttggaagaattgttgtcagttactacatctagattggaacatttgaagtcacatgttaagtacccattggaagatgaaatctctagagctttgaagcatccattgcataaggaattgaacagattgggtgcaagatactacatctcaatctatgaaaagtttgattctcataataagttgttattggaatttgctaaattagattttaatagattgcaaaagatgtatcaacatgaattggcacatttgacaagatggtggaaggatttggatttcactaataagttgccatttgctagagatagaatcgttgaaggttacttctggatcttgggcatgtacttcgaaccagaaagaaaggatgttagagaattcttgaacagagttttcgctttgatcactgttgttgatgatacatacgatgtttacggtacttttaaagaattgttgttgtttactgatgcaattgaaagatggggtacttctgatttggatcaattgccaggttacatgagaatcatctatcaagctttgatggatgtttacaaccaaatggaagaaaagttgtcaatgaaagcagattgtccaacatacagattggaattcgctatcgaaactgttaaggcaatgttcagatcttatttggaagaagctagatggtcaaaggaacattacatcccatctatggaagaatacatgacagttgcattagtttcagttggttacaagactatcttgacaaactctttcgttggtatgggtgacattgctactagagaagttttcgaatgggtttttaattcaccattaatcatcagagcttctgatttgattgcaagattaggtgacgatattggtggtcatgaagaagaacaaaagaaaggtgacgctgcaacagctatcgaatgttacatcaaggaaaaccatgttactaagcatgaagcatacgatgaattccaaaagcaaatcgataatgcttggaaagatttgaataaggaagcattgagaccatttccagttccaatgacttttattacaagagttgttcatttcactagagctatccatgttatctatgcagatttctcagatggttacacaagatctgataaggctatcagaggttacatcacttctttgttggttgatccaattccattataa

SEQ ID NO: 43 - protein, 550 aa, Alpinia oxyphylla
MEKQSVTLVRDDQGIVRKSTKYHPSVWGDYFIRNSPLNLSEESTQRMIERVEELKVQVKSMFKGTSDVLQIMNLIDSIQLLRLEYHFENEIDGALRLIYEVDDKNYGLYETSLRFRLLRQHGYNVSADTFNKFKDENGSFISILNGDAKGLLSLYNASYLATHGETILDEANNYTKSQLVSLLSELEQPLATQVSLFLEAPLCRRMKSILARKYIPIYEKEAMRSDDILELAKLDFNLLQSLHQEELKKASIWWNDLALAKSLSFTRDRIVEGYYWILSMCYEPQYSRARVMCAKAFCLLSIMDDIYDNYSILEERRLLTEAIKRWNHEAVDSLPEYIKDFYLKLLKAFEEFEAELEFNEKYRVQYLQNEFKAIAISYFEESKWCVERYVPSLDEHLRVSMITSGCSMVVCSMYLGMGEVATKEIFDWCSSFPKAMEASGVIARLLNDIRSHETEQGRDHAASTVESYMKEHGVDVKVARKKLQEIVEKAWKDLNKELLNPTPVARPIIERILNLTMSMEDIYRYIDEYTSPDNKTNGDVSLVLVESIPI

SEQ ID NO: 44 - DNA, 1653 bp, synthetic construct
  source 1..1653: mol_type = other DNA
atggaaaagcaatctgttacattggttagagatgatcaaggtattgttagaaaatctacaaagtaccatccatctgtttggggtgattattttattagaaactctccattgaacctgtctgaagaatctactcaaagaatgattgaaagagttgaagaattgaaggttcaagttaaatctatgttcaagggtacatctgatgttttgcaaattatgaatctgatcgattctatccaattgttaagattagagtaccatttcgaaaacgaaattgatggtgctttaagattaatctacgaagttgatgataagaactacggtttgtatgaaacatctttaagattcagactgttgagacaacatggttataatgtttctgctgatacttttaacaagttcaaagatgaaaacggttcttttatctctatcttaaacggtgatgctaaaggtttgttatctttatataacgcttcctatctggctacacatggtgaaacaattttagatgaagctaataactacaccaagtctcaattagtttctttgttgtctgaattggaacaaccattagctactcaagtttctttatttttggaggctccattatgtagaagaatgaaatctattctggctagaaaatacatcccaatttatgaaaaggaggctatgagatctgatgatattttggaattggctaaattggatttcaacttattgcaatctctgcatcaagaagaattaaaaaaggcttctatctggtggaatgatttggctttagctaaatctttgtcttttacaagagacagaatcgttgaaggttattattggattttgtctatgtgttacgagccacaatattctagagctagagttatgtgtgctaaagctttttgtttattgtctatcatggacgatatctatgataattactctatcttggaggaaagaagattgttaacagaagctattaagagatggaatcatgaagctgttgattctttgccagaatatattaaagacttctacttgaagctgttgaaagcttttgaagaatttgaagctgaattggaattcaatgaaaagtatagagtccaatacttgcaaaatgaattcaaagctatcgctatttcttactttgaagaatctaagtggtgtgttgaaagatatgttccatctttggatgaacatttgagagtttctatgattacttctggttgttctatggttgtttgttctatgtatttgggtatgggtgaagttgctacaaaagaaatttttgattggtgttcttccttcccaaaagctatggaagcttctggtgttattgctagattattaaatgacatcaggtcacatgaaacagaacaaggtagagatcatgctgcttctacagttgaatcttatatgaaagaacacggtgttgatgttaaagttgctagaaaaaaactgcaagaaatcgttgaaaaggcttggaaagatttgaataaagaattgttgaaccccacaccagttgctagaccaattattgaaagaattttgaacctgactatgtctatggaagatatttatagatacatcgacgaatacacatctccagataataaaacaaacggtgatgtttctttggttttggttgaatctatcccaatttaa

SEQ ID NO: 45 - DNA, 55 bp, synthetic construct
  source 1..55: mol_type = other DNA
gttggtagacccaatcccaatgtgaattgaattgaattgaaatcgatagatcaat

SEQ ID NO: 46 - DNA, 57 bp, synthetic construct
  source 1..57: mol_type = other DNA
gttggcacttcttctggtaacttccattatagttttttctccttgacgttaaagtat

SEQ ID NO: 47 - DNA, 56 bp, synthetic construct
  source 1..56: mol_type = other DNA
ctctatactttaacgtcaaggagaaaaaactataatggaagttaccagaagaagtg

SEQ ID NO: 48 - DNA, 50 bp, synthetic construct
  source 1..50: mol_type = other DNA
ttgatctatcgatttcaattcaattcaattcacattgggattgggtctac

SEQ ID NO: 49 - DNA, 59 bp, synthetic construct
  source 1..59: mol_type = other DNA
ctttgttggtagacccaatcccaatgtgaattgaattgaattgaaatcgatagatcaat

SEQ ID NO: 50 - DNA, 59 bp, synthetic construct
  source 1..59: mol_type = other DNA
aaccagaagtggatagcacatttaacgacattatagttttttctccttgacgttaaagt

SEQ ID NO: 51 - DNA, 59 bp, synthetic construct
  source 1..59: mol_type = other DNA
tactttaacgtcaaggagaaaaaactataatgtcgttaaatgtgctatccacttctggt

SEQ ID NO: 52 - DNA, 52 bp, synthetic construct
  source 1..52: mol_type = other DNA
tatcgatttcaattcaattcaattcacattgggattgggtctaccaacaaag

SEQ ID NO: 53 - DNA, 55 bp, synthetic construct
  source 1..55: mol_type = other DNA
tttgggtgaccacgtcccattctgaattgaattgaattgaaatcgatagatcaat

SEQ ID NO: 54 - DNA, 53 bp, synthetic construct
  source 1..53: mol_type = other DNA
gtctgaaagtttcaccagaagacattatagttttttctccttgacgttaaagt

SEQ ID NO: 55 - protein, 555 aa, Actaea racemosa
MEVKRRSANYKPSVWGDKFLEYSSPDALKADAKEAKKDAVTEKKLEKLSEEVAKKLVELVDKPQQALNLINEIERLGLSHHFLPEIEAALRQISVTYDELCESLSVDDLDNVALCLRILRSHGHDVSAGVFEKFMDSNGKLKESFLNDAIGLLSLYEATHYRVHGEDLLESLLSETTSLLEALKSQLKYPLKDLIELALKLPLYDLVNLLGARYYIKIYEKYSSHNKLLLEFAKLSGNRMQKQYQHELAELVRDWKDLDTENKLPFARDNIVEGYFNILGMYAEPEHIDVREFLNRVFDLLSHIDDTYVVYGTFEEVILFTNALERWEESALDQLPEDFKIIYQALMDVYSQEEEKLAKKEDAPKYRLEFAIETVKALTRSYLEIARWSKERYIPTVEEYMSVALVSCGASTILTCSFVGMGSEATREVFEWVSSSPLIVRASDLINALGRDIGSHEEEQKWGLAATYIECYMKEYGVTKQEAYAEAQKQIDNAKKDLNQEALRPFPVPREYITRVVNSTRTIRVIYADKHDGYTHPEKKIKGLIHSLLVQPIPM

SEQ ID NO: 56 - DNA, 1668 bp, synthetic construct
  source 1..1668: mol_type = other DNA
atggaagtcaagcgtagatctgctaactacaagccatctgtctggggagacaaattcttggaatactcctccccagatgccttaaaggctgatgccaaggaagctaagaaggacgctgtcactgaaaaaaagttggaaaagttgtccgaggaagtcgcgaagaagttggttgaattagttgacaagccacaacaagctttgaatctgatcaacgaaattgaaagattgggtttgtctcatcacttcctaccagaaatcgaagcagctttgagacaaatctctgttacctacgacgagttgtgcgaatctttgtctgtcgatgatttggacaacgttgctttgtgtttgagaattttgagatcccatggtcacgacgtctccgctggtgttttcgaaaagttcatggactctaacggtaagttaaaagaatccttcttgaacgatgctattggtttgttgtccttgtatgaagccacacattacagagttcacggtgaagacttgttagaatctttgttgtctgaaactacttctttgttggaagccttgaagtctcaattgaaatacccattgaaggacttgattgaattggctttgaagttgcctctgtacgatttggttaacttgttgggtgcgagatactacatcaagatatacgaaaagtactcttcacacaacaagttgttgcttgagtttgccaagctgtctggtaacagaatgcaaaagcaataccaacacgaattggccgaattggtcagagactggaaagatttggataccgaaaacaagttacctttcgctcgtgataacattgttgaaggttacttcaacatcttgggtatgtacgctgaaccagaacacattgacgtccgtgaattcttaaacagagtttttgacttgctgtcccacatcgatgacacttacgttgtttacggtactttcgaagaagttatcttgttcaccaacgctttggaaagatgggaagaatccgctttggaccaattgccagaagatttcaagatcatttaccaagctttgatggatgtctactcacaagaagaagaaaagttggctaagaaggaagacgctccaaagtacagattggaattcgccattgaaactgttaaggctctcacccgttcttacttggaaatcgccagatggtctaaggaaagatacatcccaactgtcgaagaatatatgagtgtcgccttagtgtcttgtggtgcttccactattttgacttgttctttcgttggtatgggttccgaagctaccagagaagtttttgaatgggtttcctcctctccacttatcgttagagcttctgacttaattaatgctttaggtagagatatcggttctcacgaagaagaacaaaagtggggcttagctgctacttatatcgaatgttacatgaaggaatacggtgtcaccaagcaagaagcttacgccgaagctcaaaagcaaattgacaacgctaagaaagacttgaaccaagaagctctaagaccattcccagttccaagagaatatattacccgcgttgtcaactccaccagaactatcagagtaatctacgctgacaagcacgatggttacacccacccagaaaagaaaatcaagggtttgattcactctttattggtccaaccaattccaatgtga

SEQ ID NO: 57 - DNA, 52 bp, synthetic construct
  source 1..52: mol_type = other DNA
catgatatcgacaaaggaaaaggggcctgttcacattggaattggttggacc

SEQ ID NO: 58 - DNA, 47 bp, synthetic construct
  source 1..47: mol_type = other DNA
gtaagaatttttgaaaattcaatataaatggaagtcaagcgtagatc

SEQ ID NO: 59 - protein, 555 aa, Actaea racemosa
MEVKRRSANYKPSVWGDKFLEYSSPDALKADAKEAKKDAVTEKKLEKLKEEVAKMLVETVDKPQQALNLINEIQRLGLSHHFLPEIEAALRQISVTYDELCESLSVDDLDNVALCLRILRSHGHDVSAGVFEKFMDSNGKLKGSFLNDAIGLLSLYEATHFRVHGEDLLESLLSLTTSLLEALKSQLKYPLKDEITLALKLPLYDEVNLLGARYYIKIYEKYSSHNKLLLEFAKLDGNRMQKQYQHELAELVRDWKDLDTENKLPFARDRIVEGYFNILGMYAEPEHKDVREFLNRVFDLLSHIDDTYVVYGTFEEVILFTNAIERWEESALDQLPEDMKIIYQALMDVYSQEEEKLAKKEDAPKYRLEFAIETVKALTRSYLEIARWSKERYIPTVEEYMSVALVSCGASTILTCSFVGMGDEATREVFEWVSSSPLIVRASDLINALGRDIGSHEEEQKWGLAATYIECYMKEYGVTKQEAYAEAQKQIDNAKKDLNQEALRPFPVPREYITRVVNSTRTIRVIYADKHDGYTHPEKKIKGLIHSLLVQPIPM

SEQ ID NO: 60 - DNA, 1668 bp, synthetic construct
  source 1..1668: mol_type = other DNA
atggaagttaagagaagatctgctaactacaagccttccgtctggggtgacaaattcttggaatactcttctccagatgccttgaaggctgacgctaaggaagctaagaaggatgctgtcactgaaaagaagttagagaagttgaaggaagaagtcgctaagatgttggttgaaactgttgacaagccacaacaagctttgaacttgatcaacgaaatccaaagattgggtttgtcccatcacttcttgccagaaattgaagctgccttgagacaaatctctgtaacttacgatgaattgtgtgaatccttgtctgtcgatgatttggacaacgttgctctatgtttgagaattttgagatcccatggtcacgatgtttccgctggtgtcttcgaaaagttcatggactccaacggtaagttgaagggttctttcttgaacgatgctattggtctattgtccttgtacgaagctacccatttcagggtccacggtgaagacttattggaatctttgctgtctttgaccacttctttgttggaagcactgaagtctcaattgaaatacccattgaaggacgaaatcactttggctttgaagttgccattgtacgacgaggttaatctattaggtgccagatactacatcaagatctacgaaaagtactcatcacacaacaagttgttattagaatttgccaaattggatggtaacagaatgcaaaagcaataccaacacgaattagctgaattggtccgtgactggaaggacttggacactgaaaacaaattaccatttgcaagagacagaatcgtcgaaggttacttcaacatcttgggtatgtacgctgaaccagaacacaaggacgttagagaattcttgaacagagtttttgatcttttgtctcacattgatgacacctacgttgtttacggtaccttcgaagaagtcatcttgttcaccaacgccattgaaagatgggaagaatctgccctcgaccaattaccagaagacatgaagatcatctaccaagctttgatggatgtctactcccaggaagaagaaaagttggccaagaaggaagatgctccaaagtacagattggaattcgctatcgaaaccgtcaaggccctaacaagatcttacttggaaattgctagatggtctaaggaacgttacattccaaccgttgaagaatatatgtctgttgctttagtttcttgtggtgcttccactattttgacttgctccttcgtcggtatgggtgatgaagccacccgtgaagttttcgaatgggtttctagttcccctttgattgtcagagcttctgacttgattaatgctttgggtagagatatcggttcccacgaagaagaacaaaagtggggattggctgctacttacatagaatgttacatgaaagaatatggtgttaccaagcaagaagcttacgctgaagctcaaaagcaaattgataacgctaagaaagacttgaaccaagaagccttaagaccattcccagttccaagagaatacattacccgtgttgtcaactctaccagaactatcagagtgatctatgctgacaagcacgacggctacactcacccagaaaagaagattaagggtttgattcactccttactagttcaaccaatcccaatgtga

SEQ ID NO: 61 - DNA, 51 bp, synthetic construct
  source 1..51: mol_type = other DNA
gatatcgacaaaggaaaaggggcctgttcacattgggattggttgaactag

SEQ ID NO: 62 - DNA, 46 bp, synthetic construct
  source 1..46: mol_type = other DNA
gaatttttgaaaattcaatataaatggaagttaagagaagatctgc

SEQ ID NO: 63 - protein, 555 aa, Actaea racemosa
MEVKRRSANYKPSVWGDKFLEYSSPDALKADSKEAKKDAVTEKKLEKLKEEVAKMLVETVQKPQQALNLINEIQRLGLSFHFLPEIEAALRQISVTYDELCESLSVDDLDNVALCLRILRSHGHDVSAGVFEKFMDSNGKLKGSFLNDAIGLLSLYEATHFRVHGEDLLESLLSLTTSLLEALKSQLKYPLKDEITLALKLPLYDEVNRLGARYYIKIYEKYSSHNKLLLEFAKLDGNRMQKMYQHELAELTRDWKDLDTENKLPFARDRIVEGYFNILGMYAEPEHKDVREFLNRVFDLLSHIDDTYVVYGTFEEVILFTNAIERWETSALDQLPEDMKIIYQALMDVYSQEEEKLAKKEDAPKYRLEFAIETVKALTRSYLEIARWSKERYIPTVEEYMSVALVSCGASTILTCSFVGMGDEATREVFEWVSSSPLIVRASDLINALGRDIGSHEEEQKWGLAATYIECYMKEYGVTKQEAYAEAQKQIDNAKKDLNQEALRPFPVPREYITRVVNFTRAIRVIYADKHDGYTHPEKKIKGYITSLLVQPIPM

SEQ ID NO: 64 - DNA, 1668 bp, synthetic construct
  source 1..1668: mol_type = other DNA
atggaagtcaagcggagatctgctaactacaagccatccgtctggggtgacaaatttttggaatattcatccccagacgccttgaaagctgattccaaggaagccaagaaggatgctgtcactgaaaagaaattagaaaaattaaaggaagaagttgccaagatgttggttgaaactgtccaaaagccacaacaagctttaaacttgatcaacgaaatccaaagattgggtttgtctttccactttctgccagaaattgaagccgctttgagacaaatctccgttacttacgacgaattgtgtgaatctttgtctgtcgatgacttggacaacgttgcattgtgcttgagaatcttacgttctcacggtcacgatgtttccgctggtgtattcgaaaagttcatggactctaacggtaagttaaagggttctttcttgaacgatgccattggtttattgtcattgtacgaagctactcacttcagagttcacggtgaagaccttttggaaagcctcttgtctttgaccacttccctattggaagctttgaagtcccaattgaagtacccattgaaggacgaaatcaccttggccttgaagttgccattatatgatgaagtcaacagattgggtgctagatactacatcaagatctacgaaaagtactcctctcacaacaagctgttgttggagtttgctaagctcgacggaaacagaatgcaaaagatgtaccaacacgaattagctgaattgaccagagattggaaagacttggatactgaaaacaagctacctttcgctagagacagaattgtcgaaggttacttcaacattttgggtatgtatgctgaaccagaacacaaggacgttcgtgaattcttgaatcgtgtcttcgacttgttgtctcacattgacgacacttacgttgtttacggtactttcgaagaagttatcttgttcaccaacgctatcgaaagatgggaaaccagtgccttggaccaattacctgaagacatgaaaattatctaccaagctttgatggacgtctactctcaagaagaagaaaagttggcaaagaaagaagatgctccaaagtacagattagaattcgctattgaaaccgttaaggctttaactcgttcctacttggaaatcgccagatggtctaaggaaagatacattccaaccgtcgaagaatatatgtctgtcgctttggtttcttgtggtgcctccactatcttgacctgttccttcgttggtatgggtgatgaagctacaagagaagtttttgagtgggttagctcttctccattgattgttagagcttctgatctaattaacgctttgggtagagacattggttcccatgaagaagaacaaaagtggggtttggctgctacctacatcgaatgttacatgaaggaatacggtgtcaccaagcaagaagcttacgctgaagctcaaaagcaaattgataatgctaagaaggatttgaaccaagaagccttaagaccattcccagttccaagagaatacattactagagttgttaacttcaccagagccatcagagtcatctacgctgacaagcatgatggttacacccatccagaaaaaaagattaagggttacatcacttctttattggtccaaccaatcccaatgtga

SEQ ID NO: 65 - DNA, 52 bp, synthetic construct
  source 1..52: mol_type = other DNA
catgatatcgacaaaggaaaaggggcctgttcacattgggattggttggacc

SEQ ID NO: 66 - DNA, 47 bp, synthetic construct
  source 1..47: mol_type = other DNA
gtaagaatttttgaaaattcaatataaatggaagtcaagcggagatc

SEQ ID NO: 67 - protein, 555 aa, Actaea racemosa
MEVKRRSANYKPSVWGDKFLEYSSPDALKADSKEAKKDAVTEKKLEKLKEEVAKMLVETVQKPQQALNLINEIQRLGLSFHFEPEIEAALRQISVTYDELCESLSVDDLDNVALCLRILRSHGHKVSAGVFEKFMDSNGKLKGSFLNDAIGLLSLYEATHFRVHGEDLLESLLSLTTSRLEYLKSQLKYPLEDEITRALKLPLYDEVNRLGARYYIKIYEKYDSHNKLLLEFAKLDGNRMQKMYQHELAELTRDWKDLDTENKLPFARDRIVEGYFNILGMYAEPEHKDVREFLNRVFDLISHVDDTYVVYGTFEEVILFTNAIERWETSALDQLPEDMKIIYQALMDVYSQEEEKLAKKADAPKYRLEFAIETVKALTRSYLEIARWSKERYIPTVEEYMSVALVSCGASTILTCSFVGMGDEATREVFEWVSSSPLIVRASDLINALGRDIGSHEEEQKWGLAATYVECYMKEYGVTKQEAYAEAQKQIDNAKKDLNQEALRPFPVPREYITRVVNFTRAIRVIYADKHDGYTHPEKKIKGYITSLLVQPIPM

SEQ ID NO: 68 - DNA, 1668 bp, synthetic construct
  source 1..1668: mol_type = other DNA
atggaagtcaagagaagatccgctaactacaagccatctgtctggggtgacaaattcttagaatattcctctccagacgctttgaaggctgactccaaggaagccaaaaaggatgccgttactgaaaagaaattggaaaagttaaaggaagaagttgccaagatgctggtcgaaactgttcaaaagccacaacaagcattaaacttgattaacgaaatccaaagattgggtttgtccttccacttcgaaccagaaattgaagctgccttgagacaaatctctgttacctacgatgaattgtgtgaatcattgtccgttgacgatttggataacgttgctctatgcttgagaatcttgagatctcacggtcacaaggtttccgctggtgtttttgaaaagttcatggattctaacggtaagttgaaaggttctttcttgaacgatgctattggtttgctttccttgtacgaagccactcatttcagagttcacggtgaagatttgttggaatccttgctctctctcactacttccagattggaatatttgaagtcccaattgaagtacccattggaagacgaaatcaccagagctctaaagttacctttatacgacgaagttaaccgtttgggcgccagatactacatcaagatttacgaaaagtatgactctcacaacaagttgttgttggaattcgccaaattggatggtaacagaatgcaaaagatgtaccaacacgaattagctgaattaaccagagactggaaggatttggacaccgaaaacaagttgccatttgctagagacagaattgttgaaggttacttcaacatcttgggtatgtacgctgaaccagaacacaaagacgttagagaatttttaaatcgtgtcttcgatctaatatctcacgtcgatgacacttacgtcgtctacggtactttcgaagaagtcattttgttcaccaacgccattgaaagatgggaaacctccgctttggaccaattgccagaggacatgaaaatcatctaccaagctttgatggacgtttactctcaagaagaagaaaaactggctaagaaggctgatgcccctaagtacagattggaattcgctattgaaactgtcaaggccttgacccgttcttacttggaaattgctagatggtccaaggaaagatacattccaaccgttgaagagtatatgtctgttgctctagtctcttgtggtgcttctacaatcttgacttgttctttcgttggtatgggtgatgaagctacccgtgaagtcttcgaatgggtttcttccagtccattgattgtcagagcttctgacttgatcaatgctttaggtagagatatcggtagccacgaagaagaacaaaagtggggtttggctgccacttacgtcgaatgttacatgaaggaatacggtgtcaccaagcaagaagcttacgctgaagctcaaaagcaaattgacaacgctaagaaggacttgaaccaagaagctttaagaccattcccagttccaagagaatacatcactcgtgttgtcaacttcactagagctatcagagttatctacgccgacaagcatgacggttacactcacccagaaaagaagatcaagggttacattacctctttgttggtccaaccaatcccaatgtga

SEQ ID NO: 69 - DNA, 52 bp, synthetic construct; identical to SEQ ID NO: 65
  source 1..52: mol_type = other DNA

SEQ ID NO: 70 - DNA, 49 bp, synthetic construct
  source 1..49: mol_type = other DNA
gtaagaatttttgaaaattcaatataaatggaagtcaagagaagatccg

SEQ ID NO: 71 - protein, 555 aa, Actaea racemosa
MEVKRRSANYKPSVWGDKFLEYSSPDHLKNDSDELKKDAVTEKKLEKLKEEVAKMLVETVQKPQQALNLINEIQRLGLSFHFEPEIEAALRQISVTYHELCESLNVDDLDNVALCLRILREHGHKVSAGVFEKFMDSNGKLKGSFLNDAIGLLSLYEATHFRVHGEDLLESLLSLTTSRLEYLKSQLKYPLEDEITRALKLPLYKEVNRLGARYYIKIYEKYDSHNKLLLEFAKLDGNRMQKMYQHELAELTRDWKDLDTENKLPFARDRIVEGYFNILGMYAEPECKDVREFLNRVFDLISHVDDTYVVYGTFEEVILFTNAIERWETSALDQLPEDMKIIYQALMDVYSQEEEKLAKKADAPKYRLEFAIETVKALTRSYLEIARWSKERYIPTVEEYMSVALVSCGAKTILTCSFVGMGDEATREVFEWVSSSPLIVRASDLINALGDDIGSHEEEQKWGLAATYVECYMKEYGVTKQEAYAEAQKQIDNAKKDLNQEALRPFPVPREYITRVVNFTRAIRVIYADKHDGYTHPEKKIKGYITSLLVQPIPM

SEQ ID NO: 72 - DNA, 1668 bp, synthetic construct
  source 1..1668: mol_type = other DNA
atggaagtcaagagaagatccgctaactacaagccatctgtctggggtgacaaattcttagaatactcctctccagaccacttgaagaacgattccgatgaactaaagaaggatgctgtcactgaaaagaaattggaaaagttgaaggaagaagttgctaagatgttggtcgaaacagtccaaaagcctcaacaagccttgaacttgatcaacgaaatccaaagattaggtttgtctttccactttgaaccagaaattgaagcagctttgagacaaatctccgtcacctaccacgaattgtgtgaatccctgaatgtcgatgatttggacaacgttgccttgtgtttgagaatcttgcgtgaacacggtcacaaggtttctgctggtgtcttcgaaaagttcatggactctaacggtaagttgaagggttccttcctaaacgacgctatcggtttgttgagtttgtacgaagccactcacttcagagtccatggtgaagacttgttggaatctttgttgtccttgaccacctcaagattggaatacttgaagtctcaattgaaatacccattggaagatgaaatcactagagctttaaagttacctttatacaaagaagttaaccgtttgggagctagatactatatcaagatttacgaaaagtacgattctcacaacaagttgttgttggaattcgctaaattggatggtaacagaatgcaaaagatgtaccaacacgaattagctgaactgaccagagactggaaggacctagacaccgaaaacaaattgccatttgctcgtgacagaattgttgaaggttacttcaacattctgggtatgtacgctgaaccagaatgtaaggatgttagagaattcttgaacagagttttcgatttgatttctcacgttgacgacacttacgtcgtctacggtactttcgaagaagtcatcttgttcaccaacgccattgaaagatgggaaacttctgctttggaccaattgccagaagacatgaagatcatctatcaagctttgatggatgtttactctcaagaagaagagaagttggccaagaaggctgatgctccaaagtacagactagaatttgccattgaaactgttaaagcattgaccagatcttacttggaaattgctagatggtctaaggaacgttacattccaactgttgaagaatacatgtccgttgctttggtttcttgtggtgctaagaccatcttgacttgctccttcgttggtatgggtgacgaagctacccgcgaagttttcgaatgggtttcttcttccccattgattgtcagagcttctgacttgattaatgctttgggtgatgacattggttcccatgaagaagaacaaaagtggggtttagccgctacttacgttgaatgttacatgaaagaatacggtgttaccaagcaagaagcttacgccgaagctcaaaagcaaattgacaatgccaagaaggacttaaaccaagaagctctaagaccattcccagttccaagagaatatatcactagagtcgtcaacttcactagagccattcgtgttatctatgctgacaagcacgatggctacactcatccagaaaagaagatcaagggttacatcacctctttattggttcaaccaatcccaatgtga

SEQ ID NO: 73 - DNA, 52 bp, synthetic construct
  source 1..52: mol_type = other DNA
catgatatcgacaaaggaaaaggggcctgttcacattgggattggttgaacc

SEQ ID NO: 74 - DNA, 49 bp, synthetic construct; identical to SEQ ID NO: 70
  source 1..49: mol_type = other DNA

SEQ ID NO: 75 - protein, 555 aa, Actaea racemosa
MEVKRRSANYKPSVWGDKFLEYSSPDHLKNDSDELKKDAVTEKKLEKLKEEVAKMLVETVQKPQQALNLINEIQRLGLSFHFEPEIEAALRQISVTYHELCESLNVDDLDNVALCFRILREHGHKVSAGVFHKFMDSNGKLKGSFLNDAIGLLSLYEATHFRVHGEDLLEDLLSLTTSRLEYLKSQMKYPLEDEITRALKHPLYKEVNRLGARYYIKIYEKYDSHNKLLLEFAKLDGNRMQKMYQHELAELTRDWKDLDTTNKLPFARDRIVEGYFNILGMYAEPECKDVREFLNRVFALISHVDDTYDVYGTFEEVILFTNAIERWETSALDQLPEDMKIIYQALMDVYSQEEEKLAKKADAPTYRLEFAIETVKALTRSYLEIARWSKERYIPTVEEYMSVALVSCGAKTILTCSFVGMGDEATREVFEWVSSSPLIVRASDLINALGDDIGSHEEEQKWGDAATYVECYMKEHGVTKQEAYAEAQKQIDNAKKDLNQEALRPFPVPRTYITRVVNFTRAIRVIYADKHDGYTHPEKKIKGYITSLLVQPIPM

SEQ ID NO: 76 - DNA, 1668 bp, synthetic construct
  source 1..1668: mol_type = other DNA
atggaagtgaagagaagatctgccaactacaagccttctgtctggggtgacaaattcttagaatactcttccccagaccacctcaagaacgactccgatgaattgaagaaggacgctgttactgaaaaaaaattagaaaagttgaaggaagaagtcgctaagatgttggtcgaaaccgtccaaaagccacaacaagctttgaacttaatcaacgaaatccaaagattaggtttgtctttccatttcgaaccagaaattgaagctgctttgagacaaatctctgttacttaccatgaattgtgtgaatccttgaatgtcgatgatttggacaacgttgctttatgtttcagaatcctacgtgaacacggacacaaagtttccgctggtgtcttccacaagttcatggactcaaacggtaagttgaagggttcttttttgaacgatgctattggtcttttgtccttgtatgaagccacccacttcagagtccatggtgaagatttgcttgaagacttgttatcattgaccacctccagattggaatatttgaagtctcaaatgaagtacccactggaagatgaaatcacgagagctttgaagcatccattgtacaaggaagtcaacagactaggtgccagatactacatcaagatttacgaaaagtacgattcccacaacaagttgttgttggaatttgctaaattggatggtaacagaatgcaaaagatgtaccaacacgaactggccgaattgacccgtgactggaaggatttagacaccactaacaagctaccttttgccagagacagaattgttgaaggttacttcaacattttgggtatgtatgctgaaccagaatgcaaagatgttagagaattcttgaacagagttttcgctttgatatctcacgttgatgacacttacgatgtttacggtactttcgaagaagttatcttgttcaccaacgccatcgaaagatgggaaacttctgccttggaccaattgccagaagacatgaagattatctaccaagctttgatggatgtctactcccaagaagaggaaaagttggctaagaaggctgatgctccaacctaccgtttggaattcgctatcgaaacagtcaaggctcttactaggtcttacttggaaattgctagatggtctaaggaacgttacattccaactgttgaagaatacatgtccgttgctttggtatcttgtggcgccaagaccattttgacttgttctttcgttggtatgggtgacgaggctaccagagaagtctttgaatgggtttcttcctctccattgattgtcagagcctctgacttgattaacgctttgggtgatgacatcggttcgcacgaagaagaacaaaaatggggtgacgcagctacttacgtcgaatgttacatgaaagaacacggtgtcaccaagcaagaagcttacgctgaagctcaaaagcagattgacaatgctaagaaggatctgaaccaagaagccttaagaccattcccagttccaagaacctatattactagagttgttaacttcactagagctatcagagtcatttacgctgacaagcacgacggttacactcacccagaaaagaagatcaagggttacatcacttccttgttggttcaaccaatcccaatgtga

SEQ ID NO: 77 - DNA, 52 bp, synthetic construct; identical to SEQ ID NO: 73
  source 1..52: mol_type = other DNA

SEQ ID NO: 78 - DNA, 49 bp, synthetic construct
  source 1..49: mol_type = other DNA
gtaagaatttttgaaaattcaatataaatggaagtgaagagaagatctg

SEQ ID NO: 79 - protein, 555 aa, Actaea racemosa
MEVKRRSANYKPSVWGDKFLEYSSPDHLKNDSDELKKDAVTEKKLEKLKEEVAKMLVETVQKPQQALNLINEIQRLGLSFHFEPEIEAALRQISVTYHELCESTNVDDLDNVALCFRILREHGHKVSADVFHKFMDSNGKLKGSFLNDAIGLLSLYEATHFRVHGEDLLEDLLSLTTSRLEYLKSQMKYPLEDEITRALKHPLYKELNRLGARYYISIYEKYDSHNKLLLEFAKLDGNRMQKMYQHELAELTRDWKDLDTTNKLPFARDRIVEGYFNILGMYFEPECKDVREFLNRVFALISHVDDTYDVYGTFEEVILFTHAIERWETSALDQLPEYMKIIYQALMDVYSQMEEKLAKKADAPTYRLEFAIETVKALFRSYLEIARWSKERYIPTVEEYMSVALVSCGAKTILTCSFVGMGDTATREVFEWVSSSPLIVRASDLINALGDDIGSHEEEQKWGDAATYVECYMKEHGVTKQEAYAEAQKQIDNAKKDLNQEALRPFPVPRTYITRVVNFTRAIRVIYADSHDGYTHPEKKIKGYITSLLVQPIPM

SEQ ID NO: 80 - DNA, 1668 bp, synthetic construct
  source 1..1668: mol_type = other DNA
atggaagttaagagaagatctgctaactacaagccatctgtctggggtgacaaattcttggaatactcttctccagaccacttgaagaacgactctgatgaattgaagaaggatgctgtcactgaaaagaaattggaaaaattaaaggaagaagttgccaagatgttggttgaaactgttcaaaagccacaacaagccttaaacttgatcaacgaaatccaaagactaggtttgtccttccatttcgaacctgaaattgaagctgccttgagacaaatttccgttacttaccacgaattgtgtgaatctactaacgtcgacgatttggataacgtcgctctctgtttcagaatcttacgtgaacatggtcacaaggtttccgctgatgtcttccacaagttcatggactctaacggtaagttgaagggttctttcttgaacgatgcaattggcctattatcattgtacgaagctactcacttcagagtccacggtgaagatttattggaagacttgttgagcttgactacttctagattggaatacttgaagtctcaaatgaagtatccattggaagacgaaatcaccagagctcttaagcacccattatacaaggaattgaaccgtttaggtgctcgttactacatctcgatctacgaaaagtacgattctcacaacaagttgttgctcgaattcgctaagttggacggtaacagaatgcaaaagatgtaccaacacgaattggctgaattaactagagactggaaggacttggataccaccaacaagttgccattcgctagagacagaattgtcgaaggttacttcaacattttgggtatgtattttgaacctgaatgtaaggatgttagagagttcttgaatagagtttttgccttgatttcccatgtcgacgacacttacgacgtttacggtactttcgaggaggtcatcttgttcacccacgcaattgaaagatgggaaacatctgccttagaccaattgccagaatatatgaaaatcatctaccaagctttgatggatgtctactcccaaatggaagaaaaattggccaaaaaagctgatgctccaacctacagattggaatttgctatcgaaaccgtcaaggctttgtttcgttcttacttggaaattgccagatggtctaaggaaagatacattccaactgtcgaagaatacatgtctgtggctttggtttcttgcggtgctaagaccatcttgacctgttccttcgtcggtatgggtgacactgccacgagagaagttttcgaatgggtttctagctctccattgattgttcgcgcttccgatttgatcaatgctttgggtgatgacattggttcccacgaagaagaacaaaaatggggtgacgctgctacctacgttgaatgttacatgaaggaacacggtgttaccaagcaagaagcttacgctgaagctcaaaagcaaatcgacaacgctaagaaggacttgaaccaagaagctctaagaccattcccagttccaagaacttacattaccagagttgttaacttcactcgtgccatcagagtcatttacgctgactcccacgatggttacacccatccagaaaagaagatcaagggttatattacctccttgctggtccaaccaatcccaatgtga

SEQ ID NO: 81 - DNA, 52 bp, synthetic construct; identical to SEQ ID NO: 65
  source 1..52: mol_type = other DNA

SEQ ID NO: 82 - DNA, 49 bp, synthetic construct
  source 1..49: mol_type = other DNA
taagaatttttgaaaattcaatataaatggaagttaagagaagatctgc

SEQ ID NO: 83 - protein, 555 aa, Actaea racemosa
MEVTRRSANYHPSVWGDKFLEYSSPDHLKNDSDELKNDAVTEKKLEKLKEEVKKMLVETVQKPQQALNLINEIQRLGLSFHFEPEIEAALRQISVTYHELCESTNVDDLDNVALCFRILREHGHKVSADVFHKFMDSNGKLKGSFLNDAIGLLSLYEATHFRVHGEDLLEDLLSLTTSRLEYLKSQMKYPLEDEITRALKHPLYKELNRLGARYYISIYEKYDSHNKLLLEFAKLDGNRMQKMYQHELAELTRDWKDLDFTNKLPFARDRIVEGYFNILGMYFEPECKDVREFLNRVFALISHVDDTYDVYGTFEEVILFTHAIERWETSALDQLPEYMKIIYQALMDVYSQMEEKLAKKADAPTYRLEFAIETVKALFRSYLEIARWSKERYIPTMEEYMSVALVSCGAKTILTNSFVGMGDTATREVFEWVSSSPLIVRASDLINALGDDIGGHEEEQKWGDAATAVECYMKEHGVTKQEAYAEAQKQIDNAKKDLNQEALRPFPVPMTYITRVVNFTRAIRVIYADSDDGYTHPEKKIKGYITSLLVQPIPM

SEQ ID NO: 84 - DNA, 1668 bp, synthetic construct
  source 1..1668: mol_type = other DNA
atggaagttactagaagatccgctaactatcatccatctgtctggggtgacaaattcttggaatactcttctccagaccatttgaagaatgatagcgacgaattgaagaacgacgctgtcactgaaaagaagctggaaaaacttaaggaagaagtcaagaagatgttggtggaaaccgtccaaaagccacaacaagctttgaacttgatcaacgaaatccaaagattgggtttgagtttccacttcgagcctgaaattgaagctgctttgagacaaatctctgttacctaccacgaattgtgcgaatccaccaacgtcgatgatttagacaacgttgctttgtgtttcagaattctcagagaacacggtcacaaggtttctgctgatgttttccacaagttcatggactccaacggtaagttgaagggttctttcttgaacgatgctatcggtttgttgtccttgtacgaggccacccacttccgtgtccatggtgaagacttattggaagatttgttgtctttgactacttccagattggaatacttgaaatcccaaatgaagtacccattggaagatgaaatcaccagagctttaaagcacccattgtacaaggaattaaatagattaggtgctagatactacatctcgatttacgaaaagtatgattctcacaacaaattgttgctggaattcgctaagttggatggtaacagaatgcaaaagatgtaccaacacgaattggctgaacttacacgtgactggaaggacttggacttcactaacaagctaccattcgccagagacagaatcgttgaaggttacttcaacatcttgggtatgtattttgaaccagaatgtaaggatgttagagaattcttaaacagagtttttgccttgatttcccacgttgacgacacttacgacgtctacggtactttcgaggaagttatcttgttcacccatgccattgaaagatgggaaacttctgccttggaccaattgccagaatatatgaagatcatttaccaagctttgatggacgtttactcccaaatggaagaaaagttggctaagaaggctgatgctccaacttacagattggaatttgctatcgaaactgtcaaggccttattcagatcttacttggaaattgctagatggtctaaggaacgttacattccaaccatggaagaatacatgtctgtcgctttggtttcttgtggtgccaagaccattttgactaactcattcgttggtatgggtgacactgctactcgtgaagtctttgaatgggtttcttcctcccctttgatcgtcagagcttctgacttgatcaatgctctgggtgacgatattggtggtcacgaagaagaacaaaagtggggtgatgccgctaccgccgtcgaatgttacatgaaagaacacggtgttaccaagcaagaagcttacgctgaggctcaaaagcaaattgacaacgctaagaaggatttgaaccaagaagccttaagaccattcccagttccaatgacctacattacccgtgttgttaacttcaccagagctatcagagtcatttacgctgactctgatgacggttacactcacccagaaaaaaaaatcaagggctacatcacttctttgttagttcaaccaattccaatgtga

SEQ ID NO: 85 - DNA, 52 bp, synthetic construct
  source 1..52: mol_type = other DNA
tcgacaaaggaaaaggggcctgttcacattggaattggttgaactaacaaag

SEQ ID NO: 86 - DNA, 49 bp, synthetic construct
  source 1..49: mol_type = other DNA
taagaatttttgaaaattcaatataaatggaagttactagaagatccgc

SEQ ID NO: 87 - protein, 555 aa, Actaea racemosa
MEVTRRSANYHPSVWGDKFLEYSSPDHLKNDSDHLKNDAVTEKKLEKLKEEVKKMLVETVQKPQQALNLINEIQRLGLSFHFEPEIEAALRQISVTYHELCESTNVDDLDNVALCFRILREHGHKVSCDVFHKFMDSNGKLKGSFLNDAIGLLSLYEATHFRVHGEDLLEDLLSLTTSRLEYLKSQMKYPLEDEITRALKHPLHKELNRLGARYYISIYEKYDSHNKLLLEFAKLDGNRMQKMYQHELAELTRWWKDLDFTNKLPFARDRIVEGYFNILGMYFEPECKDVREFLNRVFALISHVDDTYDVYGTFEEVILFTHAIERWETSALDQLPEYMKIIYQALMDVYSQMEEKLAKKADAPTYRLEFAIETVKALFRSYLEIARWSKERYIPTMEEYMTVALVSCGAKTILTNSFVGMGDTATREVFEWVSSSPLIVRASDLINALGDDIGGHEEEQKKGDAATAVECYMKEHGVTKQEAYAEFQKQIDNAWKDLNQEALRPFPVPMTYITRVVHFTRAIHVIYADSDDGYTHPEKKIKGYITSLLVDPIPM

SEQ ID NO: 88 - DNA, 1668 bp, synthetic construct
  source 1..1668: mol_type = other DNA
atggaagtcaccagaagatccgctaactaccatccatctgtctggggtgacaagttcttggaatactcctctccagaccatttgaaaaatgattcagaccacttgaagaacgatgctgtcactgaaaagaaattggagaaattgaaggaagaagttaagaagatgttggtcgaaactgttcaaaagccacaacaggctttgaacttgatcaacgaaatccaaagattaggtttgtccttccacttcgaacctgaaattgaagcagctttgagacaaatctctgtcacttaccacgaattgtgtgaatctaccaacgtcgatgatttggacaacgttgctctttgtttcagaatcttgagagaacatggtcacaaggtttcttgtgatgttttccataaattcatggactctaacggtaagttgaaaggttctttcttaaacgacgctatcggtttgttgtccttgtacgaagctacccacttcagagttcacggtgaagatttgttggaagacttattgtctttgaccacatccagattagaatacttgaagtctcaaatgaagtacccattggaagatgaaatcaccagagcccttaaacacccattgcacaaggaattgaacagattgggggctagatactacatctccatctatgaaaagtacgactcccacaacaagttgttgttggaatttgctaagttagatggtaacagaatgcaaaagatgtaccaacacgaactggctgaattgaccagatggtggaaggacctagacttcaccaacaagttgccattcgccagagacagaattgttgaaggttacttcaacattctcggtatgtatttcgaaccagaatgtaaggatgttagagaattcttgaaccgtgtttttgccttaatttctcacgttgatgacacttacgatgtttacggtactttcgaagaagttatcttattcacccacgccattgaaaggtgggaaacctctgctttggaccaattgccagaatatatgaagattatctaccaagctttgatggatgtctactctcaaatggaagagaagttggccaagaaggctgatgctccaacttacagattggaattcgctatcgaaaccgttaaggccttatttagatcttacttagaaattgctcgttggagtaaggaaagatacatcccaaccatggaagaatacatgactgtcgctctagtctcctgcggtgctaagactatcttgactaactcttttgtcggtatgggtgacaccgccactcgtgaagtcttcgaatgggtttcctcttctccattgattgtcagagcttcagatttgattaatgctttgggtgatgatatcggtggtcacgaagaagaacaaaagaagggtgacgctgctactgctgtcgaatgttacatgaaagaacacggtgtcaccaagcaagaagcttacgccgaattccaaaagcaaattgacaacgcttggaaggacttgaaccaagaagccttgcgtcctttcccagttccaatgacctacatcactcgtgttgtgcatttcactagagctattcacgtcatttacgctgactccgacgacggttatactcacccagaaaagaagatcaagggttacattacttctctgttggttgacccaattccaatgtga

SEQ ID NO: 89 - DNA, 52 bp, synthetic construct
  source 1..52: mol_type = other DNA
catgatatcgacaaaggaaaaggggcctgttcacattggaattgggtcaacc

SEQ ID NO: 90 - DNA, 49 bp, synthetic construct
  source 1..49: mol_type = other DNA
agtaagaatttttgaaaattcaatataaatggaagtcaccagaagatcc

SEQ ID NO: 91 - protein, 555 aa, Actaea racemosa
MEVTRRSANYHPSVWGDKFLEYSSPDHLKNDSDHLKNDAVTEKKHEKLKEEVKKMLVETVQKPQQALNLINEIQRLGLSFHFEPEIEAALRQISVTYHEYCCSTNVDDLHNVALCFRILREHGHKVSCDVFHKFMDSNGKLKGSFLNDAIGLLSLYEATHFRVHGEDLLEDLLSLTTSRLEYLKSQMKYPLEDEITRALKHPLHKELNRLGARYYISIYEKYDSHNKLLLEFAKLDGNRMQKMYQHELAELTRWWKDLDFTNKLPFARDRIVEGYFWILGMYFEPECKDVREFLNRVFALISHVDDTYDVYGTFEEVILFTHAIERWETSALDQLPEYMKIIYQALMDVYSQMEEKLAKKADCPTYRLEFAIETVKALFRSYLEIARWSKERYIPTMEEYMTVALVSVGYKTILTNSFVGMGDTATREVFEWVFSSPLIVRASDLIAALGDDIGGHEEEQKKGDAATAVECYMKEHGVTKQEAYAEFQKQIDNAWKDLNQEALRPFPVPMTYITRVVHFTRAIHVIYADSDDGYTRPEKKIKGYITSLLVDPIPM

SEQ ID NO: 92 - DNA, 1668 bp, synthetic construct
  source 1..1668: mol_type = other DNA
atggaagtcactagaagatctgctaactaccatccatctgtctggggtgacaagttcttagaatactcttctccagaccacttgaagaacgattctgaccatttgaagaacgacgctgtcaccgaaaagaagcacgaaaagttgaaagaagaagtcaagaagatgttggttgaaactgtccaaaagccacaacaagctttgaacttgatcaacgaaatccaaagattgggtttgtctttccacttcgaacctgaaattgaagcggctttgagacaaatctcagttacttaccacgaatactgttgttccactaatgtcgacgatttgcacaacgttgccctttgtttcagaattttaagagaacacggtcacaaggtttcttgcgatgttttccataaattcatggattccaacggtaagttgaagggttcctttttgaatgatgctattggtctgttgtctttgtacgaagctactcatttcagagtccacggtgaagatttgttggaagatctcttatccttgaccacttctagattggaatacttgaagtcccaaatgaaatacccattggaagatgaaatcaccagagctctaaaacacccattacacaaggaattgaaccgcttgggtgctcgttactacatttctatctacgaaaagtacgactctcacaacaaattgcttttggaatttgctaagttggatggtaacagaatgcaaaagatgtaccaacacgaattggctgaattgactagatggtggaaagacttggatttcacaaacaagttgccattcgctagagacagaatcgtggaaggttacttctggattcttggtatgtattttgaaccagaatgtaaagacgtcagagaattcttgaacagagtttttgccttgatctcccacgtcgatgatacttacgatgtctacggtactttcgaagaagttatcttgttcactcacgctattgaacgttgggaaacctctgccttagaccaattgccagaatacatgaagattatctaccaagctttgatggacgtttactctcaaatggaagaaaagttggccaagaaggctgactgtccaacctacagattggaattcgctatcgaaactgttaaggccttgtttcgtagttacttggaaattgccagatggtctaaggaaagatacatcccaaccatggaagaatatatgactgttgctttagtctccgtcggttacaagaccatcttgactaactctttcgttggtatgggtgacactgctaccagagaagtcttcgaatgggttttctcctccccattaattgttagagcttctgacttgattgctgccttgggtgatgacatcggtggacacgaagaagaacaaaagaagggtgacgctgctaccgccgtcgaatgttacatgaaggaacatggtgttaccaagcaagaagcttacgctgaattccaaaagcaaattgacaacgcttggaaggatttaaaccaagaagctttgcgtcctttcccagttccaatgacctatatcactagagttgttcacttcaccagagccattcacgttatctatgctgattccgacgacggttacaccagaccagaaaaaaagatcaagggctacatcacatccctattggttgacccaattccaatgtga

SEQ ID NO: 93 - DNA, 52 bp, synthetic construct; identical to SEQ ID NO: 89
  source 1..52: mol_type = other DNA

SEQ ID NO: 94 - DNA, 49 bp, synthetic construct
  source 1..49: mol_type = other DNA
taagaatttttgaaaattcaatataaatggaagtcactagaagatctgc

SEQ ID NO: 95 - protein, 572 aa, Actaea racemosa
MSLLVLSTSGSAPLTKKLEVKRRSANYKPSVWGDKFLEYQSPDALKADAEEAKKDAVEEKKLEKLSEEVAKMLVEHVHKPQQALNLINEIERLGLSHHFLPEIEAALRQISVTYEELCRSLSVDDLSNVALCLRILREHGHDVSASVFTKFMDSNGKLKASFLNDAIGLLSLYEATHFRVAGEDLLESLLSLTTSLLEALKSQLKYPLKDEIRMALKSPLAKEINRLGARYYIKIYEKYSSHNKLLLEFAILDGNRMQKQYQRELAELTRDWKDLDTDNKLPFARDNIVSGFFLIYGMYSEPEMKDVREFLNRVFDLISHVDDYYTVYGTFEEVILFTEAFERWTWSALDQLPEDMKIIFQALMDVYSQEEEKLAKKDDAPKYRLEFAIETVKALTRSLLEIARWSKEREIPTLEEYMKVALVSCGFKTILTCSFVGMGTRATREVFEWVSSSPLIVRASELIAMLGDDIGAHEEEQKEGDAATAIECYMKEYGVTKEEAYAEFQKEIDEAWKDLNQEALRPFPVPWSYIDRVVNLTRAWHRIYADDHDGYTYPEKKIKGWINSLFHTPIPA

SEQ ID NO: 96 - DNA, 1719 bp, synthetic construct
  source 1..1719: mol_type = other DNA
atgtctctcttggtcttgtccacatccggttctgctccattgaccaagaagttggaagtcaagagaagatctgctaactacaagccatctgtctggggtgacaagttcttggagtaccaatctccagacgcattgaaggctgacgctgaagaagctaagaaagatgctgtcgaagaaaagaagttggaaaaattgtctgaagaagttgctaagatgttggttgaacacgtccacaagccacaacaagctttgaatttgatcaacgaaattgaacgtttgggtttgtctcatcactttttgccagaaatcgaagccgccttgagacaaatttccgtcacttacgaagaattgtgtcgttctttgagtgtcgacgacttatctaacgttgctttatgcttgagaatcctgcgtgaacacggtcacgatgtctccgcctctgttttcaccaaattcatggactccaacggtaagttgaaggcttctttcttgaacgatgctatcggtttgctttccttgtacgaagctactcatttcagagttgccggtgaagatttgttggaatctttattgtctttgaccacttccttgttagaagccttgaagtcccaattgaagtacccattgaaagatgaaatcagaatggctttgaagtcccctctggccaaggaaatcaacagattgggtgctagatactacatcaagatctacgaaaagtactcctctcacaacaagttattgttggaattcgccattttggatggtaacagaatgcaaaagcaataccaaagagaattggctgaattaaccagagactggaaggacctagacactgacaacaagttgccatttgccagagataacatcgtctctggtttcttcttgatttacggcatgtactctgaaccagaaatgaaggatgtcagagagttcttaaatagagtcttcgacctgatctcccacgttgatgactattacactgtttacggtacctttgaagaagttatcttgttcactgaagctttcgaaagatggacctggtctgccttggaccaattaccagaagacatgaaaatcatcttccaagctttgatggatgtctactctcaagaagaagaaaagctcgctaaaaaggatgatgctccaaagtacagattggaattcgctattgaaaccgttaaggctttgaccagatccttgctcgaaatcgctagatggtccaaggaaagagaaatcccaactttggaagaatatatgaaggttgctttagtttcttgtggtttcaagaccatcttgacttgttctttcgttggtatgggtactcgtgctaccagagaagtcttcgaatgggtttcatcttctcctttgattgtcagagcttccgaattgatcgctatgttgggtgacgatattggtgctcacgaagaagaacaaaaggaaggtgatgctgcaactgccattgaatgttacatgaaggaatacggtgttaccaaggaagaagcttacgctgaatttcaaaaggaaattgacgaagcctggaaagatttgaaccaagaagccctcagaccattcccagttccatggtcttacattgaccgtgttgttaacttgactagagcttggcacaggatttatgctgacgaccatgacggttacacctacccagaaaagaagattaagggttggattaactctttattccacactccaattccagcttga

SEQ ID NO: 97 - DNA, 52 bp, synthetic construct
  source 1..52: mol_type = other DNA
catgatatcgacaaaggaaaaggggcctgttcaagctggaattggagtgtgg

SEQ ID NO: 98 - DNA, 48 bp, synthetic construct
  source 1..48: mol_type = other DNA
gtaagaatttttgaaaattcaatataaatgtctctcttggtcttgtcc

SEQ ID NO: 99 - protein, 572 aa, Actaea racemosa
MSLLVLSTSGSAPLTKSLEVKRRSANYKPSVWGDKFLEYSSPDALKADAEEAKKDAVEEKKLEKLKEEVAKMLVETVHKPQQALNLINEIQRLGLSHHFLPEIEAALRQISVTYEELCRSLSVDDLSNVALCLRILREHGHDVSASVFTKFMDSNGKLKASFLNDAIGLLSLYEATHFRVAGEDLLESLLSLTTSLLEALKSQLKYPLEDEIRRALKSPLAKEINRLGARYYIKIYEKYSSHNKLLLEFAILDGNRMQKQYQRELAELTRDWKDLDFDNKLPFARDNIVEGFFLIYGMYSEPEMKDVREFLNRVFDLISHVDDYYTVYGTFEEVILFTEAFERWTWSALDQLPEDMKIIFQALMDVYSQEEEKLAKKADAPKYRLEFAIETVKALTRSLLEIARWSKERYIPTMEEYMKVALVSCGFKTILTCSFVGMGTRATREVFEWVSSSPLIVRASELIAMLGDDIGAHEEEQKEGDAATAIECYMKEYGVTKQEAYAEFQKQIDNAWKDLNQEALRPFPVPWSYIDRVVNLTRAWHRIYADDHDGYTYPEKKIKGWITSLFVTPIPA

SEQ ID NO: 100 - DNA, 1719 bp, synthetic construct
  source 1..1719: mol_type = other DNA
atgtctctattggtcttgtctacctctggttctgctccattgactaagagcttagaagtcaagagaagatccgctaactacaagccatctgtctggggtgacaagtttttggaatatagctctccagatgctttaaaggctgatgctgaagaagccaagaaggatgctgttgaagaaaaaaaattagaaaagttgaaggaagaagtggctaagatgttggtggaaactgtccacaagccacaacaagctctgaacttgatcaacgaaatccaaagattgggtctatcccatcatttcttgccagaaattgaagctgctttgcgtcaaatttccgttacttacgaagaattatgcagatctttgtcagtcgatgatttgtccaacgttgctttgtgtttgcgtattttgagagaacacggtcacgatgtctctgcttccgtcttcaccaagttcatggattctaacggtaagttaaaggcttctttcttgaatgacgctattggtttgttgtctttgtacgaagctacccacttcagagtcgctggtgaagacttgttggaatctttgctcagtttgactacctccttgttggaagcccttaaatctcaattgaaatacccattggaagatgaaatcagaagagccttgaagtctccattggctaaggaaatcaaccggttaggtgccagatactacattaagatttacgaaaagtactcatctcacaacaagttgttactcgaattcgccatattggatggtaacagaatgcaaaagcaataccaaagagaattggctgaattgacacgtgactggaaggatctagatttcgataataagttgccttttgccagagacaacattgtcgaaggtttcttcttgatttatggtatgtactctgaaccagaaatgaaggacgttagagaatttttgaacagagttttcgacttgatctcccatgttgacgactactacaccgtttacggtactttcgaagaagttatcctattcactgaagccttcgaaagatggacctggtccgccttggaccaattgccagaggacatgaaaatcatcttccaagccttgatggacgtctactcccaagaagaagaaaagctagctaagaaggctgacgccccaaagtacagattggaattcgctattgaaactgtcaaagctttgaccagatctttattggaaatcgctcgttggtctaaggaaagatacattccaaccatggaagaatatatgaaggttgctttggtttcttgtggtttcaagaccatcttgacttgttccttcgttggtatgggtaccagagctactagggaagtttttgaatgggtttcctcttcccctctgatcgtcagagcctccgaattgattgctatgttgggcgatgacatcggtgctcacgaagaagaacaaaaagaaggtgatgctgctactgctatcgaatgttacatgaaggaatacggtgttaccaagcaagaagcttacgccgaattccaaaaacaaattgacaacgcttggaaggacttgaaccaagaagcattaagaccattcccagttccatggtcttacatcgacagagttgttaacctaactagagcttggcacagaatctacgctgacgaccacgacggttacacctacccagaaaagaagatcaagggttggattacttctttgttcgtcactccaatcccagcttga

SEQ ID NO: 101 - DNA, 51 bp, synthetic construct
  source 1..51: mol_type = other DNA
catgatatcgacaaaggaaaaggggcctgttcaagctgggattggagtgac

SEQ ID NO: 102 - DNA, 51 bp, synthetic construct
  source 1..51: mol_type = other DNA
gtaagaatttttgaaaattcaatataaatgtctctattggtcttgtctacc

SEQ ID NO: 103 - protein, 572 aa, Actaea racemosa
MSLLVLSTSGSAPLTKSSEVKRRSANYKPSVWGDKFLEYSSPDALKADSEEAKKDAVEEKKLEKLKEEVAKMLVETVQKPQQALNLINEIQRLGLSHHFLPEIEAALRQISVTYEELCRSLSVDDLSNVALCFRILREHGHDVSASVFTKFMDSNGKLKGSFLNDAIGLLSLYEATHFRVAGEDLLESLLSLTTSRLEALKSQLKYPLEDEITRALKSPLAKEINRLGARYYIKIYEKYSSHNKLLLEFAILDGNRMQKQYQRELAELTRDWKDLDFDNKLPFARDRIVEGFFLIYGMYSEPEMKDVREFLNRVFDLISHVDDTYTVYGTFEEVILFTEAFERWTWSALDQLPEDMKIIYQALMDVYSQEEEKLAKKADAPKYRLEFAIETVKALTRSLLEIARWSKERYIPTMEEYMKVALVSCGYKTILTCSFVGMGTRATREVFEWVSSSPLIVRASELIAMLGDDIGAHEEEQKEGDAATAIECYMKEYGVTKQEAYAEFQKQIDNAWKDLNQEALRPFPVPWSYITRVVNLTRAWHRIYADDHDGYTYPEKKIKGWITSLFVTPIPA

SEQ ID NO: 104 - DNA, 1719 bp, synthetic construct
  source 1..1719: mol_type = other DNA
atgtctttgttggtcttgtccacttccggttcagctccattgactaaatcttctgaagtcaagagaagatccgctaactacaagccatccgtctggggtgacaagttcttagaatatagttctccagacgccctcaaagctgattctgaggaagccaaaaaggatgctgtcgaagaaaagaaattggaaaagttgaaggaagaggtcgctaagatgttggttgaaaccgttcaaaagccacaacaagctttgaatttaattaacgaaatccaacgtttgggtttgagccatcacttcttgcctgaaatcgaagctgctttaagacaaatctccgttacctacgaagaattgtgcagatccttgtctgtcgatgatttatccaacgttgctttgtgtttcagaatcttgagagaacacggtcacgatgtctccgcctctgtctttaccaagttcatggacagtaacggtaagttgaagggttctttcttgaacgacgctatcggtttgttatccttgtacgaagctacccatttcagagtcgctggtgaagacttgttggaatctttgttgtctttaacaacttccagattggaagctttgaagtctcaattgaaatacccattggaagatgaaattactagagctctaaaatctccactagccaaggaaattaatcggttaggtgccagatactacattaagatctatgaaaagtactcttcccacaacaagcttttgctagaatttgctattctagatggtaacagaatgcaaaagcaataccaacgtgaattggctgaattgacccgtgactggaaggacttggatttcgacaacaagttgccttttgccagagacagaattgttgaaggcttcttcctgatttacggtatgtactctgaaccagaaatgaaggatgtcagagaatttttgaaccgtgttttcgatttgatctctcacgttgacgacacttacaccgtctacggtactttcgaagaagttattttattcactgaagctttcgaaagatggacctggtctgctttggaccaattgccagaagacatgaaaatcatctaccaagctttgatggatgtctactcccaagaagaagaaaagttagctaagaaggctgacgccccaaagtacagattggaattcgccattgaaactgttaaggccttgacccgttcgttacttgaaatcgctagatggtccaaggaacgttacatcccaaccatggaagaatacatgaaggttgctttggtttcttgtggttacaagaccatcctgacttgttctttcgttggtatgggtaccagagctaccagagaagtcttcgaatgggtttcctcctccccattaattgttagagcctctgaattgatcgctatgttgggtgatgacattggtgctcacgaagaagaacaaaaggaaggtgatgctgccactgctattgaatgttacatgaaggaatacggtgttaccaagcaagaagcttacgctgaattccaaaaacaaattgacaacgcttggaaggacttgaaccaagaagctttaagaccattcccagttccatggtcttacatcactagagttgttaacttgacaagagcttggcacagaatctacgcagatgaccacgacggttacacttatccagaaaagaagatcaagggttggatcacctctttgttcgtgactccaattccagcttga

SEQ ID NO: 105 - DNA, 51 bp, synthetic construct
  source 1..51: mol_type = other DNA
catgatatcgacaaaggaaaaggggcctgttcaagctggaattggagtcac

SEQ ID NO: 106 - DNA, 48 bp, synthetic construct
  source 1..48: mol_type = other DNA
gtaagaatttttgaaaattcaatataaatgtctttgttggtcttgtcc

SEQ ID NO: 107 - protein, 572 aa, Actaea racemosa
MSLLVLSTSGSAPLTKSSEVKRRSANYKPSVWGDKFLEYSSPDALKADSDEAKKDAVEEKKLEKLKEEVAKMLVETVQKPQQALNLINEIQRLGLSHHFEPEIEAALRQISVTYHELCRSLSVDDLSNVALCFRILREHGHDVSASVFTKFMDSNGKLKGSFLNDAIGLLSLYEATHFRVHGEDLLESLLSLTTSRLEALKSQLKYPLEDEITRALKHPLAKEINRLGARYYIKIYEKYDSHNKLLLEFAILDGNRMQKMYQRELAELTRDWKDLDFTNKLPFARDRIVEGFFLIYGMYSEPEMKDVREFLNRVFDLISHVDDTYTVYGTFEEVILFTEAFERWEWSALDQLPEDMKIIYQALMDVYSQEEEKLAKKADAPKYRLEFAIETVKALTRSLLEIARWSKERYIPTMEEYMKVALVSCGYKTILTCSFVGMGTRATREVFEWVSSSPLIVRASELIAMLGDDIGAHEEEQKEGDAATAIECYMKEYGVTKQEAYAEFQKQIDNAWKDLNQEALRPFPVPWSYITRVVNLTRAIHRIYADDHDGYTYPEKKIKGYITSLFVTPIPA

SEQ ID NO: 108 - DNA, 1719 bp, synthetic construct
  source 1..1719: mol_type = other DNA
atgtccctgttggtcttgtctacttctggttccgctccattgactaagtcttccgaagttaagagaagatctgctaactacaagccatctgtctggggtgacaaattcttggaatactcttctccagacgccttgaaagccgattctgacgaagctaagaaagatgccgtcgaagaaaagaagttggaaaagttgaaggaagaagtcgctaagatgttggtagaaactgtccaaaagccacaacaagcgcttaacttgattaacgaaatccaaagattgggtttgtcccatcactttgaaccagaaattgaagctgctttgagacaaatctccgttacttaccacgaattatgtcgttctttgtctgttgacgatctttcaaacgttgccttgtgtttcagaattctacgtgaacacggtcacgacgttagtgcttccgttttcaccaagttcatggattccaatggaaagctcaagggttctttcttgaacgatgccattggtttattgtccttgtacgaggctactcatttcagagtccacggtgaagatttgttagaatccttgttgtctttgactacctccagattggaagccttgaagtcccaattgaagtacccattggaagatgaaatcactagagctttgaagcacccattggccaaggaaatcaaccgtttgggcgctcgttactacatcaagatttacgaaaaatacgattctcacaacaaattgttgttggaatttgctatcttggacggtaacagaatgcaaaagatgtaccaaagagaattggctgaactgacaagagactggaaggatttggatttcaccaacaagttacctttcgccagagacagaatcgttgaaggtttcttcttgatctacggtatgtactcagagccagaaatgaaggatgtcagagaattcttaaatagagttttcgacttgatctctcatgttgatgacacttacactgtttacggtactttcgaagaagtcatcttattcactgaagctttcgaaagatgggaatggtctgctctcgaccaattgccagaagacatgaagattatttaccaggctttgatggacgtctacagtcaagaagaagaaaaattagcaaagaaggctgatgctccaaagtacagattggaattcgctatcgaaaccgtcaaggctctaactagatccttgttggaaattgctcgttggtccaaggaaagatatattccaaccatggaagaatatatgaaggttgctttagtctcttgtggttataagaccattttgacctgctctttcgtcggtatgggtaccagagctacccgtgaagtttttgaatgggtttcctcctctcctttgatcgttagagcttctgaattaatcgctatgttaggtgatgacatcggtgctcacgaagaagaacaaaaggaaggtgacgccgccactgctattgaatgttacatgaaagaatacggtgttaccaagcaagaagcttacgcagaattccaaaagcaaattgacaacgcttggaaggacttgaaccaagaagctttaagaccattcccagttccatggtcttacattaccagagttgtcaacttgaccagagccattcacagaatctacgctgacgaccacgatggttacacgtacccagaaaagaagattaagggttacatcacctctttgtttgttactccaatcccagcttga

SEQ ID NO: 109 - DNA, 53 bp, synthetic construct
  source 1..53: mol_type = other DNA
catgatatcgacaaaggaaaaggggcctgttcaagctgggattggagtaacaa

SEQ ID NO: 110 - DNA, 47 bp, synthetic construct
  source 1..47: mol_type = other DNA
gtaagaatttttgaaaattcaatataaatgtccctgttggtcttgtc

SEQ ID NO: 111 - protein, 572 aa, Actaea racemosa
MSLLVLSTSGSAPTTKSSEVKRRSANYKPSVWGDKFLEYSSPDALKADSDEAKKDAVTEKKLEKLKEEVAKMLVETVQKPQQALNLINEIQRLGLSFHFEPEIEAALRQISVTYHELCRSTNVDDLSNVALCFRILREHGHDVSADVFTKFMDSNGKLKGSFLNDAIGLLSLYEATHFRVHGEDLLESLLSLTTSRLEALKSQLKYPLEDEITRALKHPLAKEINRLGARYYIKIYEKYDSHNKLLLEFAILDGNRMQKMYQHELAELTRDWKDLDFTNKLPFARDRIVEGFFLIYGMYSEPEMKDVREFLNRVFDLISHVDDTYDVYGTFEEVILFTEAFERWEWSALDQLPEDMKIIYQALMDVYSQEEEKLAKKADAPKYRLEFAIETVKALTRSLLEIARWSKERYIPTMEEYMKVALVSVGYKTILTNSFVGMGTRATREVFEWVSSSPLIVRASELIAMLGDDIGAHEEEQKKGDAATAIECYMKEYGVTKQEAYAEFQKQIDNAWKDLNQEALRPFPVPWSYITRVVNFTRAIHRIYADDHDGYTYPEKKIKGYITSLFVTPIPA

SEQ ID NO: 112 - DNA, 1719 bp, synthetic construct
  source 1..1719: mol_type = other DNA
atgtctttgttagttttgtccacatctggtagcgctccaactaccaagtcttccgaagttaagagaagatctgctaactacaagccaagtgtctggggtgacaagtttttagagtacagctctccagacgctttgaaagccgactccgatgaagccaaaaaggacgctgtcactgaaaagaagttggaaaaattgaaggaagaagttgccaagatgttggtcgaaactgttcaaaagccacaacaagctttgaacttgatcaacgaaatccaaagacttggtttgtccttccacttcgaaccagaaatcgaagctgccttaagacaaatatccgttacctaccatgaattatgtcgttccaccaacgttgatgatttgtcaaatgtcgccttgtgtttcaggatcttgagagaacacggtcacgacgtctctgccgatgtctttactaaattcatggactccaacggtaagttgaagggttctttcttgaacgatgctattggtctactgtctttgtacgaagccactcatttcagagtccatggtgaagatttgttggaatctttgttgtcattgaccacttccagactagaggctctgaagtcccaattgaagtatccattagaagacgaaattaccagagctttgaagcacccattggctaaggaaataaaccgtttgggtgccagatactacatcaagatttacgaaaagtacgactcccacaacaagttattgttggaattcgctatcttggacggtaacagaatgcaaaagatgtaccaacacgaattggcagaattgaccagagactggaaggatttggatttcaccaacaagcttccttttgccagagacagaattgttgaaggtttcttcttgatttacggtatgtactctgaaccagaaatgaaagatgttagagaattcttgaatagagttttcgacttgatctctcacgttgacgacacttacgatgtctacggtacttttgaagaagtcattttgttcactgaagctttcgaaagatgggaatggagtgctttggaccaattaccagaagacatgaagatcatttaccaagctttgatggatgtttattctcaagaagaagaaaagttggctaagaaggctgacgccccaaagtacagattagaatttgccattgaaaccgtcaaggctttgaccagatccttgttggaaatcgctagatggtctaaggaacgttacattccaaccatggaagaatacatgaaggttgctttggtgtctgttggttacaagaccatcttaactaactctttcgtcggtatgggtacccgtgctacccgtgaagttttcgaatgggtttcttcttccccattgattgtcagagcttctgaattaattgctatgttgggcgacgatatcggtgctcacgaagaagaacaaaagaagggtgatgctgctactgctatcgaatgttacatgaaggaatatggtgtcaccaagcaagaagcatatgctgaattccaaaagcaaattgacaacgcttggaaggacttgaaccaagaagctttaagaccattcccagtcccatggtcttacatcactagagttgttaacttcactagagctattcacagaatctacgctgatgaccacgatggttacacttacccagaaaagaaaatcaaaggttacattacgtctttgttcgttactcctatcccagcttga

SEQ ID NO: 113 - DNA, 52 bp, synthetic construct
  source 1..52: mol_type = other DNA
catgatatcgacaaaggaaaaggggcctgttcaagctgggataggagtaacg

SEQ ID NO: 114 - DNA, 50 bp, synthetic construct
  source 1..50: mol_type = other DNA
gtaagaatttttgaaaattcaatataaatgtctttgttagttttgtccac

SEQ ID NO: 115 - protein, 572 aa, Actaea racemosa
MSLLVLSTSGSAPTTKSSEVKRRSANYKPSVWGDKFLEYSSPDALKNDSDELKKDAVTEKKLEKLKEEVAKMLVETVQKPQQALNLINEIQRLGLSFHFEPEIEAALRQISVTYHELCRSTNVDDLSNVALCFRILREHGHKVSADVFTKFMDSNGKLKGSFLNDAIGLLSLYEATHFRVHGEDLLEDLLSLTTSRLEYLKSQMKYPLEDEITRALKHPLAKEINRLGARYYIKIYEKYDSHNKLLLEFAILDGNRMQKMYQHELAELTRDWKDLDFTNKLPFARDRIVEGYFLIYGMYFEPEMKDVREFLNRVFDLISHVDDTYDVYGTFEEVILFTEAFERWEWSALDQLPEDMKIIYQALMDVYSQEEEKLAKKADAPKYRLEFAIETVKALTRSYLEIARWSKERYIPTMEEYMKVALVSVGYKTILTNSFVGMGDRATREVFEWVSSSPLIVRASELIAMLGDDIGAHEEEQKKGDAATAIECYMKEYGVTKQEAYAEFQKQIDNAWKDLNQEALRPFPVPWSYITRVVNFTRAIHRIYADSHDGYTYPEKKIKGYITSLFVTPIPA

SEQ ID NO: 116 - DNA, 1719 bp, synthetic construct
  source 1..1719: mol_type = other DNA
atgtctttgctagtcttgtctacttctggttctgctccaactactaagtcctccgaagttaagagaagatctgctaactacaagccatctgtctggggtgacaagttcttggaatactcttctccagacgctttaaagaacgactccgatgaactgaagaaggatgctgtcactgaaaagaagttggaaaaattgaaggaagaagttgctaagatgttggtcgaaactgttcaaaagccacaacaagctttaaacttgattaacgaaatccaaagattgggtttgagcttccacttcgaaccagaaatcgaagctgctttgagacaaatctctgtcacttaccacgaattgtgtcgttccaccaacgtcgatgatttgtccaatgttgctttatgtttcagaatcttgcgtgaacacggtcacaaggtcagtgccgatgttttcaccaaattcatggactccaacggtaagttgaagggttctttcttgaacgatgccattggtttgttgtctttgtacgaagctacccatttcagagttcacggtgaagacttgctagaagatttattgtccttgaccacttccagactggaatatttgaagtctcaaatgaaatatccattagaggacgaaatcactagggctttgaagcacccattggccaaggaaatcaaccggttgggtgccagatactacatcaagatttacgaaaagtacgactctcacaacaagttgttgttggaatttgctattttggatggtaacagaatgcaaaaaatgtaccaacacgaattagctgaattgaccagagactggaaagacttagatttcaccaataaattacctttcgctagagatagaatcgttgaaggttacttcttaatatatggtatgtactttgaaccagaaatgaaggacgttagagaattcttgaacagagttttcgacttgatctcccatgttgacgacacttacgatgtttacggtacctttgaagaagttatcttattcactgaagctttcgaaagatgggaatggtctgccttggaccaattgccagaagacatgaagatcatttaccaagccttgatggatgtctactcccaagaagaagaaaagttggctaagaaggctgacgctccaaagtacagattggaatttgccattgaaaccgtcaaggctctaaccagatcttacttggaaatcgctcgttggtccaaggaacgttacatcccaaccatggaagaatatatgaaggttgccttggtttctgttggttacaagactatcttgactaactcttttgtcggtatgggtgacagagctactagagaagtcttcgaatgggtttcctcttctccattgattgtcagagcttctgaattgattgctatgttgggcgatgacattggtgctcacgaagaagaacaaaagaagggtgatgctgccacagctattgaatgttacatgaaagagtacggtgttaccaagcaagaagcttacgctgaattccaaaagcaaattgacaacgcttggaaggacttgaaccaagaagccttaagaccattcccagttccatggtcttacataaccagagttgtcaacttcaccagagccattcacagaatttacgcagattctcatgacggttacacttaccctgaaaagaaaatcaaaggttacattacttcactattcgttactccaatcccagcttga

SEQ ID NO: 117 - DNA, 52 bp, synthetic construct
  source 1..52: mol_type = other DNA
catgatatcgacaaaggaaaaggggcctgttcaagctgggattggagtaacg

SEQ ID NO: 118 - DNA, 50 bp, synthetic construct
  source 1..50: mol_type = other DNA
gtaagaatttttgaaaattcaatataaatgtctttgctagtcttgtctac

SEQ ID NO: 119 - protein, 572 aa, Actaea racemosa
MSLNVLSTSGSAPTTKSSEVTRRSANYKPSVWGDKFLEYSSPDALKNDSDELKKDAVTEKKLEKLKEEVAKMLVETVQKPQQALNLINEIQRLGLSFHFEPEIEAALRQISVTYHELCRSTNVDDLSNVALCFRILREHGHKVSADVFTKFMDSNGKLKGSFLNDAIGLLSLYEATHFRVHGEDLLEDLLSLTTSRLEYLKSQMKYPLEDEITRALKHPLAKEINRLGARYYIKIYEKYDSHNKLLLEFAILDGNRMQKMYQHELAELTRDWKDLDFTNKLPFARDRIVEGYFLIYGMYFEPECKDVREFLNRVFALISHVDDTYDVYGTFEEVILFTEAFERWEWSALDQLPEYMKIIYQALMDVYSQMEEKLAKKADAPTYRLEFAIETVKALTRSYLEIARWSKERYIPTMEEYMKVALVSVGYKTILTNSFVGMGDRATREVFEWVSSSPLIVRASDLIAMLGDDIGAHEEEQKKGDAATAVECYMKEHGVTKQEAYAEFQKQIDNAWKDLNQEALRPFPVPWSYITRVVNFTRAIHRIYADSHDGYTYPEKKIKGYITSLFVTPIPM

SEQ ID NO: 120 - DNA, 1719 bp, synthetic construct
  source 1..1719: mol_type = other DNA
atgtcattaaacgtcctctctacttctggttctgccccaactactaagtcatctgaagttactagaagatctgctaactacaagccatctgtctggggtgacaagttcttggagtattcctctccagacgctttgaagaacgactccgatgaattgaagaaagatgccgtcactgaaaaaaagttggaaaagttgaaggaagaagtcgctaagatgttggttgaaaccgttcaaaagccacaacaagccttgaacttgatcaacgaaatccaaagattgggattgtctttccactttgaaccagaaattgaagccgctttgagacaaatctccgttacttaccacgaattatgcagatccactaatgtcgatgatttgtctaacgttgctttgtgtttcagaatcctaagagaacatggtcacaaggtttctgctgatgtttttaccaagttcatggactccaacggtaagctaaaaggttccttcttaaacgatgctatcggtttgttgtctttgtacgaagctactcatttcagagttcacggtgaagatttgttggaagacttgttgtctctgactacttccagactagaatacttgaagtcccaaatgaagtaccctttggaagacgaaatcacacgtgctttgaagcacccattagccaaggagatcaacagattgggtgcccgttactacatcaagatttacgaaaaatacgattcccacaacaagctgttgcttgaatttgctatcttggacggtaacagaatgcaaaaaatgtaccaacacgaattggctgaattaaccagggattggaaggatttggatttcaccaacaaattgccattcgctagagacagaattgtggaaggttacttcttgatttacggtatgtattttgaacctgaatgtaaggacgtccgtgaattcttgaatcgtgttttcgctttgatctctcatgttgacgacacttacgacgtttacggtactttcgaagaagtcattttattcactgaagctttcgaaagatgggaatggagcgcattggaccaattgccagaatacatgaaaatcatctatcaagctttgatggatgtctactctcaaatggaagaaaaattggctaagaaggctgatgctccaacctacagattagagtttgccatcgaaactgttaaggccttgaccagatcttacctagaaattgccagatggtccaaggaaagatacatcccaaccatggaagaatatatgaaggttgctttagtttccgtcggttacaagaccatcttgactaactctttcgtcggtatgggcgacagagccacccgtgaagttttcgaatgggttagttcttccccattgattgtcagagcttctgacttgattgctatgttgggtgatgacattggtgctcacgaagaagaacaaaagaagggtgacgctgctaccgctgtcgaatgttacatgaaggaacacggtgttaccaagcaagaagcttacgctgaattccaaaagcaaattgacaacgcttggaaggacttgaaccaagaagctttaagaccattcccagttccatggtcctacatcaccagagttgtcaacttcaccagagctattcacagaatctacgctgactctcacgatggttacacttacccggaaaagaagatcaagggttacattacctctttgttcgtcaccccaattccaatgtga

SEQ ID NO: 121 - DNA, 52 bp, synthetic construct
  source 1..52: mol_type = other DNA
catgatatcgacaaaggaaaaggggcctgttcacattggaattggggtgacg

SEQ ID NO: 122 - DNA, 50 bp, synthetic construct
  source 1..50: mol_type = other DNA
gtaagaatttttgaaaattcaatataaatgtcattaaacgtcctctctac

SEQ ID NO: 123 - protein, 572 aa, Actaea racemosa
MSLNVLSTSGSAPTTKSSEVTRRSANYHPSVWGDKFLEYSSPDALKNDSDELKNDAVTEKKLEKLKEEVKKMLVETVQKPQQALNLINEIQRLGLSFHFEPEIEAALRQISVTYHELCRSTNVDDLSNVALCFRILREHGHKVSADVFHKFMDSNGKLKGSFLNDAIGLLSLYEATHFRVHGEDLLEDLLSLTTSRLEYLKSQMKYPLEDEITRALKHPLAKEINRLGARYYISIYEKYDSHNKLLLEFAKLDGNRMQKMYQHELAELTRDWKDLDFTNKLPFARDRIVEGYFLIYGMYFEPECKDVREFLNRVFALISHVDDTYDVYGTFEEVILFTHAFERWETSALDQLPEYMKIIYQALMDVYSQMEEKLAKKADAPTYRLEFAIETVKALFRSYLEIARWSKERYIPTMEEYMKVALVSVGYKTILTNSFVGMGDTATREVFEWVSSSPLIVRASDLIAMLGDDIGAHEEEQKKGDAATAVECYMKEHGVTKQEAYAEFQKQIDNAWKDLNQEALRPFPVPWTYITRVVHFTRAIHRIYADSHDGYTYPEKKIKGYITSLFVTPIPM

SEQ ID NO: 124 - DNA, 1719 bp, synthetic construct
  source 1..1719: mol_type = other DNA
atgtctttgaacgtgttgtccacttctggttccgccccaactactaagtcttctgaagttaccagaagatccgctaactaccacccatctgtctggggtgacaagtttttagaatacagctccccagatgccttgaagaatgactctgacgaattgaagaacgacgctgttactgaaaagaaactagaaaagctaaaagaagaagtcaagaagatgttggttgaaactgttcaaaagccacaacaagctttgaacttaatcaacgaaatccaaagattgggtttgtctttccatttcgaaccagaaattgaagccgctttgagacaaatctccgtcacttaccatgaactttgccgttctaccaatgttgacgacttgtcaaacgttgccttgtgtttccgtatcttgagagaacacggtcacaaggtttctgctgatgttttccacaagttcatggactctaacggtaagttgaagggttctttcttgaacgatgccattggtttgttgtccttgtacgaagctacccacttcagagttcatggtgaagacttgttggaagatttattgtccttgactacctctagattggaatacttgaaatcccaaatgaaataccctttggaagatgaaatcaccagagccttaaagcatccattggccaaggaaattaacagattgggcgctagatactacatttctatctacgaaaagtacgactcccacaacaaattgcttttggaatttgctaagttggacggtaacagaatgcaaaagatgtaccaacacgaattggctgaattgacaagagactggaaggacttggatttcactaacaagctgccattcgccagagacagaattgtcgaaggttacttcttaatttacggtatgtattttgaaccagagtgtaaggacgtcagagaattcttgaacagagtcttcgctttgatctctcacgttgatgacacttacgatgtttacggtactttcgaagaagtcatcttgtttactcacgctttcgaaaggtgggaaacctctgcactagaccaattgcctgaatacatgaaaatcatctaccaagctttgatggatgtctactctcaaatggaagaaaagttggctaaaaaggctgatgctccaacctacagattagaattcgctatcgaaactgttaaggccttattcagatcttacttggaaatcgctagatggtctaaggaacgttacatcccaaccatggaagaatatatgaaggttgctttggtttctgtcggttacaagactattttgaccaactccttcgttggtatgggtgacaccgctacccgtgaagttttcgaatgggttagttcctccccattgattgttagagctagtgatttgattgctatgttgggtgacgatattggtgctcacgaagaggaacaaaagaagggtgatgctgctactgctgtcgaatgttacatgaaggaacacggtgttaccaagcaagaagcttacgctgaattccaaaagcaaattgacaacgcttggaaggatttgaaccaagaagcgttaagaccattcccagttccatggacttatatcacccgtgttgtccacttcaccagagctattcacagaatctatgctgactcacacgatggttacacttacccagaaaaaaagatcaagggttacataacttccctctttgttactccaattccaatgtga

SEQ ID NO: 125 - DNA, 52 bp, synthetic construct
  source 1..52: mol_type = other DNA
tatcgacaaaggaaaaggggcctgttcacattggaattggagtaacaaagag

SEQ ID NO: 126 - DNA, 48 bp, synthetic construct
  source 1..48: mol_type = other DNA
gtaagaatttttgaaaattcaatataaatgtctttgaacgtgttgtcc

SEQ ID NO: 127 - protein, 572 aa, Actaea racemosa
MSLNVLSTSGSAPTTKSSEVTRRSANYHPSVWGDKFLEYSSPDHLKNDSDHLKNDAVTEKKLEKLKEEVKKMLVETVQKPQQALNLINEIQRLGLSFHFEPEIEAALRQISVTYHELCRSTNVDDLHNVALCFRILREHGHKVSCDVFHKFMDSNGKLKGSFLNDAIGLLSLYEATHFRVHGEDLLEDLLSLTTSRLEYLKSQMKYPLEDEITRALKHPLHKELNRLGARYYISIYEKYDSHNKLLLEFAKLDGNRMQKMYQHELAELTRWWKDLDFTNKLPFARDRIVEGYFLIYGMYFEPECKDVREFLNRVFALISHVDDTYDVYGTFEEVILFTHAFERWETSALDQLPEYMKIIYQALMDVYSQMEEKLAKKADAPTYRLEFAIETVKALFRSYLEIARWSKERYIPTMEEYMKVALVSVGYKTILTNSFVGMGDTATREVFEWVSSSPLIVRASDLIAMLGDDIGGHEEEQKKGDAATAVECYMKEHGVTKQEAYAEFQKQIDNAWKDLNQEALRPFPVPWTYITRVVHFTRAIHVIYADSDDGYTYPEKKIKGYITSLFVDPIPM

SEQ ID NO: 128 - DNA, 1719 bp, synthetic construct
  source 1..1719: mol_type = other DNA
atgtctcttaatgtcttgtccacttctggttctgctccaaccaccaagtcttctgaagttaccagaagatccgctaactaccatccatctgtctggggtgacaagttcttggaatattcctctccagaccacttgaagaacgactcagatcatttgaagaacgatgctgtcactgaaaaaaaattggaaaagctgaaggaagaagttaagaagatgttggttgaaactgttcaaaagccacaacaagctttgaacttgatcaacgaaatccaaagattgggtttgtctttccacttcgaaccagaaattgaagctgctttgcgtcaaatctctgtcacgtaccacgaattgtgcagatctaccaacgtcgatgacttgcacaacgttgctttgtgtttcagaatcttacgtgaacacggtcacaaggtttcctgtgatgttttccataagttcatggattccaacggtaagttaaagggttccttcttgaacgatgccatcggtttgttgagcttgtacgaagctacccacttcagagttcacggtgaagacttattggaagaccttctatctttgactacctctagattagaatacttgaagtcccaaatgaagtaccctctcgaagatgaaatcacaagagctttgaagcacccattgcacaaggaattgaaccgtttgggtgcccgttactacatctccatttacgaaaagtacgattctcacaacaagttgttgttggaatttgctaagttggacggtaacagaatgcaaaagatgtaccaacacgaattggccgaactaactagatggtggaaggacttggatttcactaacaaattgcctttcgctagagacagaattgttgaaggttatttcttgatctacggtatgtacttcgaaccagaatgtaaggatgttagagaattcttaaatagagttttcgccttgatctcccacgtcgatgacacctacgacgtctatggtactttcgaagaagtcattttgttcactcacgctttcgaaagatgggaaacctctgctctcgaccaattgccagaatatatgaagattatttaccaagctttgatggatgtctactctcaaatggaagaaaagttggccaagaaagctgacgctccaacttacagactagagtttgctatcgaaactgtcaaggccttatttaggtcttacttggaaattgccagatggtctaaggaaagatacattccaaccatggaagaatacatgaaggtcgctttagtatctgttggttacaagaccatcttgaccaactctttcgtcggtatgggtgacactgctaccagagaagtctttgaatgggttagttcctccccattgattgtcagagcttctgacttgattgctatgcttggcgacgacattggtggtcacgaagaagaacaaaagaaaggtgacgctgccacggctgttgagtgttacatgaaggaacatggtgttactaagcaagaagcttacgctgaattccaaaagcaaattgacaacgcttggaaagatttgaaccaagaagcattaagaccattcccagttccatggacttacattacccgtgttgtccatttcaccagagccattcacgttatctacgccgattccgatgatggttacacttacccagaaaaaaagatcaagggttacatcacttccttatttgttgacccaatcccaatgtga

SEQ ID NO: 129 - DNA, 55 bp, synthetic construct
  source 1..55: mol_type = other DNA
gatatcgacaaaggaaaaggggcctgttcacattgggattgggtcaacaaataag

SEQ ID NO: 130 - DNA, 50 bp, synthetic construct
  source 1..50: mol_type = other DNA
gtaagaatttttgaaaattcaatataaatgtctcttaatgtcttgtccac

SEQ ID NO: 131 - protein, 572 aa, Actaea racemosa
MSLNVLSTSGSAPTTKSSEVTRRSANYHPSVWGDKFLEYSSPDHLKNDSDHLKNDAVTEKKHEKLKEEVKKMLVETVQKPQQALNLINEIQRLGLSFHFEPEIEAALRQISVTYHEYCCSTNVDDLHNVALCFRILREHGHKVSCDVFHKFMDSNGKLKGSFLNDAIGLLSLYEATHFRVHGEDLLEDLLSLTTSRLEYLKSQMKYPLEDEITRALKHPLHKELNRLGARYYISIYEKYDSHNKLLLEFAKLDGNRMQKMYQHELAELTRWWKDLDFTNKLPFARDRIVEGYFLIYGMYFEPECKDVREFLNRVFALISHVDDTYDVYGTFEEVILFTHAIERWETSALDQLPEYMKIIYQALMDVYSQMEEKLAKKADCPTYRLEFAIETVKALFRSYLEEARWSKERYIPTMEEYMTVALVSVGYKTILTNSFVGMGDTATREVFEWVFSSPLIVRASDLIARLGDDIGGHEEEQKKGDAATAVECYMKEHGVTKQEAYAEFQKQIDNAWKDLNQEALRPFPVPMTYITRVVHFTRAIHVIYADSDDGYTRPEKKIKGYITSLLVDPIPM

SEQ ID NO: 132 - DNA, 1719 bp, synthetic construct
  source 1..1719: mol_type = other DNA
atgtctttgaacgtattgtcaacttctggttccgctccaaccaccaagtctagtgaagtcaccagaagatctgctaactaccacccatccgtctggggtgacaagttcttggaatactcctctccagaccatttgaagaacgattccgaccacttgaagaacgatgctgtcactgaaaagaagcacgaaaaactcaaggaagaagttaagaagatgttggttgaaaccgttcaaaagccacaacaagctttgaacttgatcaacgaaatccaaagattaggtttgtctttccacttcgaaccagaaatcgaagctgccttgagacaaatctctgttacctaccatgaatactgttgttccaccaacgtggatgacttacacaacgttgctttgtgtttcagaattttgcgtgaacacggtcataaggtttcctgtgatgtcttccacaagttcatggactctaacggtaaattgaagggttctttcttgaacgacgctattggcttgctgagcttgtacgaagctacccactttagagttcacggtgaagatttgttggaagatctactaagtttaaccacctccagattagaatacttaaaatctcaaatgaaatacccattagaggatgaaattactcgtgctttgaagcatccattgcacaaggaattaaaccgtttgggtgctagatactacatttcaatttacgaaaagtacgattctcacaacaagttgttgttggaattcgctaagttggacggtaaccggatgcaaaagatgtaccaacacgaattggctgaattgacccgttggtggaaggacttggatttcactaataaactgcctttcgccagagacagaatcgttgaaggttacttccttatttacggtatgtatttcgaaccagaatgcaaggatgttagagaattcttgaatagagtcttcgctttgatctcccacgtcgatgacacttacgacgtttatggtactttcgaagaagttatcttgtttacccacgctatcgaaagatgggaaacttctgcattggaccaattaccagaatacatgaagatcatctaccaagctttgatggatgtctactctcaaatggaagagaagttggccaagaaagctgactgtccaacttacagattggaatttgccattgaaaccgtcaaggctcttttcagatcctacttggaagaagccagatggtctaaagaaagatatattcctaccatggaagaatatatgactgttgccttggtttctgttggttacaagaccatcttgactaactctttcgtcggtatgggtgacactgctacaagagaagtctttgaatgggttttctcttccccattgattgtcagagcttctgacttgattgctagattgggtgatgacattggtggtcacgaagaagaacaaaagaagggtgatgctgctactgccgtcgaatgttacatgaaggaacacggtgttactaagcaagaagcttacgctgaattccaaaagcaaattgacaacgcttggaaggacttaaaccaagaagccttaagaccattcccagttccaatgacttacatcactagagttgtccatttcacgagagctatccacgttatctacgccgattccgacgatggttacactcgtccagaaaagaagatcaagggttacattacctctttgttagttgacccaatcccaatgtga

SEQ ID NO: 133 - DNA, 51 bp, synthetic construct
  source 1..51: mol_type = other DNA
catgatatcgacaaaggaaaaggggcctgttcacattgggattgggtcaac

SEQ ID NO: 134 - DNA, 50 bp, synthetic construct
  source 1..50: mol_type = other DNA
gtaagaatttttgaaaattcaatataaatgtctttgaacgtattgtcaac

SEQ ID NO: 135 - protein, 548 aa, Citrus maxima
MRKKETERPTADFKPSLWRNKFLKGAKDFKTVDREATAERLEALKEEVRRMITDEEDKPVQGLRLIDEVKRLGVAYHFEKEIADALQKLSPEYIESNSPDLATVSLAFRLLRQGGIKISADVFEKFYDDAGRFKSSLINDVQGLLSLYEAAYCAVLGESILDEAIAFTTKHLKELVAQDALTPKLQEQINQALARPERQTLPLLEARYFRSFIQKSSDAKYNKTLLNFAILDHNILLELHKEELNELTKWWKELDFSKKLPYARDRLVAIYFFCLGMEAEPQYAFGREIVTRLDTILSHIHDYYFFYGTLEELELFTEAVQRWESEAISTLPEDMKLIYRELLDAFNEIEESMAKQGRSWLVEYAKEAFQKVVGAYFILAKWASEGYVPTIEEYMPIALISNAMQFVITVSFLGMGDFATKEVFEWISSMPKVVKAASIIGLLLDDMQGHEFGQKIGSWASAIECYTKQHGVSKEEAIKAFEEEVANARKQINAELMKKPQVVARPLLGLILNLARAITFIYAEDDGYFHSKLIKDQIASVLGDELPF

SEQ ID NO: 136 - DNA, 1647 bp, synthetic construct
  source 1..1647: mol_type = other DNA
atgagaaagaaggaaaccgaaagaccaaccgctgacttcaagccatctttatggagaaacaagttcttgaagggtgccaaggactttaagactgttgaccgggaagctactgctgaaagattggaagctttgaaggaggaagtcagaagaatgattaccgatgaagaggacaagccagttcaaggtttgagattgatcgatgaagtaaagagattgggtgttgcttaccatttcgaaaaggaaattgctgatgctttgcaaaaattgagcccagaatacattgaatctaactctccagacttggccactgtctccttggctttcagattattgagacaaggtggtatcaagatttctgctgatgttttcgaaaaattctacgatgatgccggtagattcaagtccagtttgattaatgatgtccaaggtttgctttcattgtacgaagctgcctactgtgctgtcttaggtgaatccatcttggacgaagctattgccttcaccactaagcatttgaaggagttagttgctcaagatgctttgactccaaagctacaagaacaaatcaaccaagctctagccagaccagaacgtcaaactttgcctttgttggaagcaagatactttagatccttcatccaaaagtcttctgacgctaagtacaacaagaccctcttgaacttcgccatcttggaccacaacatcctattggaattgcacaaggaagaattgaacgaactgaccaaatggtggaaggaactcgatttctccaagaagttgccatacgctagagacagattggtcgccatctatttcttctgtttgggtatggaagctgaaccacaatacgcttttggtcgtgaaattgttaccagattagacaccatcttgtctcacattcacgactactacttcttttacggtactttggaagaattggaattgttcactgaagccgttcaaagatgggaatctgaagctatctctaccctgccagaagacatgaaattaatctatagagaattgttggacgctttcaacgaaatcgaagaatccatggctaaacaaggtagatcttggttggttgaatatgctaaagaagctttccaaaaggttgttggtgcttacttcattttggctaagtgggcttccgaaggttacgttccaactattgaagaatacatgccaatcgctttgatttccaacgctatgcaattcgttatcactgtctctttcttaggtatgggtgacttcgctaccaaggaagtctttgaatggatttcttccatgccaaaggtcgtcaaggctgcttccatcattggtttgttgttggatgacatgcaaggtcacgaattcggtcaaaagatcggctcctgggcttctgccatcgaatgttacactaagcaacacggtgtctctaaagaagaggctattaaggctttcgaagaagaagttgctaacgccagaaagcaaatcaatgccgaattgatgaagaagcctcaagttgtcgctcgtccattgttgggtttgattttaaacttggctagagctatcacattcatctacgctgaagatgatggttacttccactctaagttgatcaaggaccaaattgcttctgtcttgggagacgaattgccattctga

SEQ ID NO: 137 - DNA, 52 bp, synthetic construct
  source 1..52: mol_type = other DNA
catgatatcgacaaaggaaaaggggcctgttcagaatggcaattcgtctccc

SEQ ID NO: 138 - DNA, 50 bp, synthetic construct
  source 1..50: mol_type = other DNA
gtaagaatttttgaaaattcaatataaatgagaaagaaggaaaccgaaag

SEQ ID NO: 139 - protein, 548 aa, Citrus maxima
MRKKETERPTADFKPSLWRNHFLKGAKDFKTVDREATAERLEALKEEVRRMITDEEDKPVQGLRLIDEVKRLGVAYHFEKEIADAIQKLSPEYIESNSPDLATVSLAFRLLRQGGIKISADVFEKFYDDEGRFKSSLINDVQGLLSLYEAAYMAVRGESILDEAIAFTTTHLKELVAQDALTPKLAEQINQALARPERQTLPLLEARYFRSFIQSSSDAKYNKTLLNFAILDHNILLELHKEELNELTKWWKELDFSKKLPYARDRLVALYFFDLGMEFEPQYAFGRKIVTRLDTILSHIHDYYFFYGTLEELELFTEAVQRWESEAISTLPEDMKLIYRELLDAFNEIEESMAKQGRSWLVRYAKEAFQKVVGAYFILAKWASEGYVPTIEEYMPIALISNAMQFVITVSFLGMGDFATKEVFEWISSNPKVVKAASVIGLLLDDMQGHEFGQKIGSWASAIECYTKQHGVSKEEAIKAFEEEVANARKQINAELMKKPQVVARPLLGTILNLARAITFIYAEDDGYFHSKLIKDQIASVLGDELPF

SEQ ID NO: 140 - DNA, 1647 bp, synthetic construct
  source 1..1647: mol_type = other DNA
atgagaaagaaagaaaccgaaagaccaactgcggatttcaagccatctttgtggagaaaccacttcttgaagggtgctaaggatttcaagactgtcgacagagaagccaccgctgaacgtttggaagctttgaaagaagaagtcagaagaatgattactgatgaagaagacaagccagttcaaggtttgagattgattgacgaagttaagagattaggtgtcgcttaccatttcgaaaaggaaatcgctgacgctatccaaaagttgtctccagaatacattgaatccaactccccagacctagctactgtctctttggccttccgtttgttgagacaaggtggtatcaagatttctgccgatgtcttcgaaaagttctacgatgacgaaggtagattcaaatcatcccttattaacgatgttcaaggtttgttatccttgtacgaagctgcttacatggccgttagaggtgaatctatcctagacgaagctatagcttttaccacgactcatttgaaggaattggttgctcaagatgctttgactccaaagttggccgaacaaatcaaccaagctttagctcgtccagaaagacaaactttaccattgttggaagccaggtatttcagatctttcatccaatcctcctctgacgccaagtacaacaagaccttattgaacttcgccattttggaccacaacatcctcttggaattgcacaaggaagaattgaatgaattgaccaagtggtggaaggaattggatttctctaagaagttgccatacgctcgtgacagattagttgctttgtatttcttcgacttgggtatggaattcgaaccacaatacgcctttggtcgaaaaattgtcaccagattggacactatcttgtctcacattcacgactactacttcttttacggtactttggaagagttggaactcttcacagaagctgtccaaagatgggaatctgaagctatttctactctgcctgaagacatgaaattgatttacagagaattattggatgcttttaacgaaattgaagaatccatggctaagcaaggtagatcctggttggtgagatacgctaaggaagcctttcaaaaggtcgttggtgcctacttcattttggctaaatgggcttccgaaggttacgttccaaccatcgaagaatatatgccaatcgctttgatctctaatgctatgcaattcgtcatcaccgtctctttcttaggtatgggtgacttcgctaccaaggaagttttcgaatggatttcttctaacccaaaggttgtcaaggctgcttctgtcattggtctattgttggatgatatgcaaggtcacgaattcggtcaaaagatcggttcttgggcttctgctatcgaatgttacactaagcaacacggtgtttccaaggaagaagctatcaaggcctttgaagaagaagttgctaacgccagaaagcaaatcaacgctgaattgatgaagaagcctcaagttgttgccagaccattgttgggtaccatcttaaacttggctagagctatcactttcatctacgctgaagatgacggttacttccacagcaaattaatcaaggaccaaattgcttccgttttgggcgatgaattgccattctga

SEQ ID NO: 141 - DNA, 51 bp, synthetic construct
  source 1..51: mol_type = other DNA
catgatatcgacaaaggaaaaggggcctgttcagaatggcaattcatcgcc

SEQ ID NO: 142 - DNA, 50 bp, synthetic construct
  source 1..50: mol_type = other DNA
gtaagaatttttgaaaattcaatataaatgagaaagaaagaaaccgaaag

SEQ ID NO: 143 - protein, 548 aa, Citrus maxima
MRKKETERPTADFKPSLWRNHFLKGAKDFKTVDREATAERLEALKEEVRRMITDEEDKPVQGLRLIDEVKRLGVAYHFEKEIADAIQKLSPEYIHSNSPDLATVSLAFRLLRQGGIKISADVFEKFYDDEGRFKSSLINDVQGLLSLYEAAYMAVRGESILDEAIAFTTTHLKSLVAQDALTPKLAEQINQALARPERQTLPLLEARYFRSFIQSTSDALYNKTLLNFAILDFNILLELHKEELNELTKWWKELDFSKKLPYARDRLVALYFFDLGMEFEPQYAFGRKIVTRLNTILSHIDDYYFFYGTLEELELFTEAVQRWNSEAISTLPEDMKLIYRELLDAFNEIEESMAKQGRSWLVRYAKEAFQKVVGAYFVLAKWASEGYVPTIEEYMPIALISNAMQFVITVSFLGMGDFATKEVFEWISSNPKVVKAASVIGLLLDDMQGHEFGQKIGSWASAIECYTKQHGVSKEEAIKAFEEEVANARKQINAELMKKPQVVARPLLGTILNLARAITFIYAEDDGYTHSYLIKDQIASVLGDELPF

SEQ ID NO: 144 - DNA, 1647 bp, synthetic construct
  source 1..1647: mol_type = other DNA
atgagaaagaaggaaaccgaaagaccaactgctgactttaaaccatctttgtggagaaaccacttcttgaagggtgccaaggatttcaagactgtcgatcgtgaagctaccgctgaaagattggaagctttgaaagaagaagtccgcagaatgattactgacgaggaagacaagccagttcaaggtttgagattaatcgacgaagttaagagattaggtgttgcttaccatttcgaaaaagagattgccgacgctatccaaaagctgtctccagaatacattcacagcaactccccagacttggctactgtttctttggctttcagattactaagacaaggtggtatcaagatctccgctgatgtcttcgaaaagttctatgatgacgaaggtagattcaagtcctctctaattaacgatgttcaaggtttgttgtccttgtacgaagctgcttacatggctgttagaggcgaatctatcttagacgaagccattgcattcaccactactcatttgaagtctttggttgctcaagatgctttgactccaaagttggctgaacaaattaaccaagctttggcaagaccagaacgtcaaactttgccattgttggaagcccgttacttcagatctttcattcaatccacctctgatgccttgtacaacaagaccttgttgaacttcgccatattggacttcaacatcttattggaattgcacaaggaagaattgaatgaattgaccaagtggtggaaggaactggacttctctaagaaactcccatacgccagagacagattggtcgctctatattttttcgatttgggtatggaatttgaaccacaatacgccttcggtagaaagatcgttaccagattgaacactatcttgtctcacattgacgactactacttcttctacggtactttggaagaattagaattgttcactgaagcagtccaaagatggaactctgaagctatctctaccttgccagaagatatgaaattaatttacagagaattgttggacgcttttaacgaaatcgaagaatccatggccaaacaaggtcgttcctggttagtaagatacgctaaggaagctttccaaaaggttgttggtgcttacttcgttttggctaaatgggctagtgaaggttacgttccaaccattgaagaatatatgccaattgctttgatttcaaatgctatgcaattcgtcatcaccgtctctttcttgggtatgggtgattttgctacgaaggaagtcttcgaatggatttcttccaaccctaaggtcgtcaaggctgcttctgttatcggtttgttattggatgacatgcaaggtcacgaattcggtcaaaagattggatcctgggcttctgctattgaatgttacaccaagcaacacggtgtctccaaggaggaagctatcaaggcctttgaagaagaagttgctaacgccagaaagcaaatcaacgccgaattgatgaagaagcctcaagttgtcgctcgtccattattgggtaccatcttgaacttggccagagctatcactttcatctacgctgaagacgatggttacactcactcttacttgatcaaggaccaaattgcttccgtcttgggtgacgaactaccattctga

SEQ ID NO: 145 - DNA, 52 bp, synthetic construct
  source 1..52: mol_type = other DNA
catgatatcgacaaaggaaaaggggcctgttcagaatggtagttcgtcaccc

SEQ ID NO: 146 - DNA, 50 bp, synthetic construct; identical to SEQ ID NO: 138
  source 1..50: mol_type = other DNA

SEQ ID NO: 147 - protein, 548 aa, Citrus maxima
MRKKETFRPTADFKPSLWRNHFLKGAKDFKTVDRTATQERLEALKEEVRRMITDEEDKPVQGLRLIDEVQRLGVAYHFEKEIEDAIQKLSPEYIHSNSPDLATVSLAFRLLRQGGIKISADVFEKFYDDEGRFKSSLINDVQGLLSLYEAAYMAVRGESILDEAIAFTTTHLKSLVAQDALTPKLAEQINQALARPERQTLPLLEARYFRSFIQSTSDALYNKTLLNFAILDFNILLELHKEELNELTKWWKELDFSKKLPYARDRLVALYFFDLGMEFEPQYAFGRKIVTRLNYILSHIDDYYFFYGTLEELELFTEAVQRWNSEAISTLPEDMKLIYRELLDAFNEIEESMAKQGRSWLVRYAKEAFQKVVGAYFVLAKWASEGYVPTIEEYMPIALTSCAMTFVITVSFLGMGDFATKEVFEWISDNPKVVKAASVIGLLLDDMQGHEFGQKIGSVASAIECYTKQHGVSKEEAIKAFEEEVANARKQINAELMKKPQVVARPLLGTILNLARAITFIYAEDDGYTHSYLIKDQIASVLGDELPF

SEQ ID NO: 148 - DNA, 1647 bp, synthetic construct
  source 1..1647: mol_type = other DNA
atgagaaagaaagaaactttcagaccaactgctgactttaaaccatccttatggagaaaccacttcttgaagggtgctaaggatttcaagactgttgacagaactgctactcaagaaagattggaagctttgaaagaagaagttagaagaatgattactgatgaagaagacaagcctgttcaaggtttgagattgattgatgaagttcaaagattgggtgtcgcttaccatttcgaaaaggaaatcgaagatgctatccaaaagttgtctccagaatacattcactccaactccccagacttggccaccgtttcattggctttccgtttgctaagacaaggtggtattaagatctctgctgatgttttcgaaaagttctacgatgacgaaggtagattcaaatcttctttgatcaacgacgtccaaggtttgttgagcttatacgaagctgcttacatggctgttagaggtgaatctatcctcgacgaagctatcgctttcaccaccactcatttgaagtctttagttgctcaagatgctctaaccccaaagttggccgaacaaattaaccaagctttggctagaccagaaagacaaactttgccattgttagaagcccgttacttcagatccttcattcagtccacttccgacgctttgtacaacaagaccctgcttaacttcgccatcttggatttcaacattttattggaattacacaaggaagaattgaacgaattgaccaagtggtggaaggaattggacttctctaagaaattgccatacgctcgtgacagattggttgccctctatttcttcgatttgggtatggaatttgaaccacaatacgcgtttggtagaaagattgtcaccagattgaactacatcttgtctcacattgacgactactactttttctacggtactttggaagaattagagttgttcactgaagctgtccaaagatggaactctgaagccatctctaccttgccagaagatatgaaactaatttacagagaattattggacgccttcaatgaaattgaagaatccatggctaaacaaggccgttcttggttggtcagatacgccaaggaagctttccaaaaggttgttggtgcttatttcgttttggctaagtgggcttctgaaggttacgttccaaccatcgaagaatatatgccaatcgctcttacatcatgtgctatgactttcgtcatcactgtctctttcttgggtatgggtgactttgctaccaaggaagtctttgaatggattagtgacaacccaaaggtcgtcaaggccgcctctgttatcggtttgttattggacgacatgcaaggtcacgaattcggtcaaaagattggttccgttgctagcgctattgaatgttacaccaagcaacacggtgtttccaaggaagaagcaatcaaggctttcgaagaagaagtcgctaacgccagaaagcaaatcaatgctgaattgatgaagaagcctcaagttgtcgcgcgtccattgttgggtaccattttaaacttggccagagctattaccttcatctacgctgaagatgatggttacactcactcttacttgatcaaggaccaaatcgcttctgtcttgggtgatgaattgccattctga

SEQ ID NO: 149 - DNA, 52 bp, synthetic construct
  source 1..52: mol_type = other DNA
catgatatcgacaaaggaaaaggggcctgttcagaatggcaattcatcaccc

SEQ ID NO: 150 - DNA, 53 bp, synthetic construct
  source 1..53: mol_type = other DNA
gtaagaatttttgaaaattcaatataaatgagaaagaaagaaactttcagacc

SEQ ID NO: 151 - protein, 548 aa, Citrus maxima
MRSKETFRPTADFKPSLWRNHFLKGAKDFKTVDRTATQERHEALKEEVRRMITDAEDKPVQGLRLIDEVQRLGVAYHFEKEIEDAIQKLSPEYIHSNSPDLATVSLAFRLLRQGGIKISADVFEKFYDDEGRFKSSLINDVQGLLSLYEAAYMAVRGESILDEAIAFTTTHLKSLVAQDALTPKLAEQINQALARPERQTLPLLEARYFRSFIQSTSDALYNKTLLNFAILDFNILLELHKEELNELTKWWKELDFTKKLPYARDRLVALYFFDLGMEFEPQYAFGRKIVTRLNYILSIIDDYYFFYGTLEELELFTEAVQRWNSEAIDTLPEDMKLIYRELLDAFNEIEEDMAKQGRSHLVRYAKEAFQKVVGAYFVLAKWASEGYVPTIEEYMPIALTSCAMTFVITVSFLGMGDFATKEVFEWISDNPKVVKAASVIGLLLDDMQGHEFGQKIGHVASAIECYTKQHGVSKEEAIKAFEEEVANARKDINAELMKKPQVVARPLLGTILNLARAITFIYKEDDGYTHSYLIKDQIASVLGDELPF

SEQ ID NO: 152 - DNA, 1647 bp, synthetic construct
  source 1..1647: mol_type = other DNA
atgagatccaaggaaactttcagaccaactgctgattttaagccatctttgtggagaaaccacttcttgaagggtgctaaggatttcaagactgttgacagaaccgctactcaagaaagacacgaagccttgaaggaagaagtcagaagaatgatcactgacgctgaagacaagccagttcaaggtttgcgtttgattgacgaagttcaaagattgggtgtcgcttatcatttcgaaaaggaaatcgaagatgccatccaaaaattgtccccagaatacattcactccaactctccagatttggctaccgtctccttagccttccgtctattgaggcagggtggtatcaagatttctgctgacgttttcgaaaagttctacgatgacgaaggtagattcaagtcttctttgatcaacgacgtacaaggtttgttatctttgtacgaagctgcttacatggctgttagaggtgagtccatcttagatgaagccattgctttcaccaccactcatttgaagtccttggttgctcaagatgctttgactccaaagttggctgaacaaatcaaccaagctttggcacgtcctgaaagacaaactttgccattgttggaagctagatatttcagatccttcattcaatcaacctccgatgctttatacaacaagaccttgttgaactttgctattctagacttcaacatcttgctggaattgcataaggaagaattaaatgaattgactaagtggtggaaggaactagatttcacaaaaaaattgccatacgctagagacagattagttgctttatacttcttcgatttgggtatggaattcgaaccacaatacgccttcggcagaaagatcgtcaccagattgaactacatcttgtctattatcgatgactactacttcttttacggtactttggaagaattggaattgttcaccgaagctgtccaaagatggaacagcgaagctatcgacaccttaccagaagacatgaaattaatttacagagaacttttggacgccttcaacgaaattgaagaagacatggccaagcaagggcgttctcacttggtgagatacgctaaggaggctttccaaaaggtcgtcggtgcttactttgtcttggccaaatgggctagtgaaggttacgttccaaccattgaagaatatatgccaattgctctaacttcttgtgctatgactttcgttatcactgtctctttcttgggtatgggtgacttcgctacgaaggaagtcttcgaatggatttctgacaacccaaaggttgttaaggctgcttctgtcatcggtctgctgttggatgatatgcaaggtcacgaatttggtcaaaagattggtcacgttgcctctgcgatagaatgttacactaagcaacacggtgtttctaaggaagaagccatcaaagcttttgaagaagaagttgccaacgccagaaaggacattaatgctgaattgatgaaaaagcctcaagttgtcgctagaccactcttaggaaccatcttgaacttggccagagctattaccttcatctacaaggaagacgatggttacacccactcatacttgatcaaggaccaaatcgcttccgttttgggtgatgaattgccattctga

SEQ ID NO: 153 - DNA, 52 bp, synthetic construct; identical to SEQ ID NO: 149
  source 1..52: mol_type = other DNA

SEQ ID NO: 154 - DNA, 50 bp, synthetic construct
  source 1..50: mol_type = other DNA
gtaagaatttttgaaaattcaatataaatgagatccaaggaaactttcag

SEQ ID NO: 155 - protein, 548 aa, Citrus maxima
MRSKETFRPTADFKPSLWRNHFLKGASDFKTVDHTATQERHEALKEEVRRMITDAEDKPVQGLRLIDEVQRLGVAYHFEKEIEDAIQKLSPNYIHSNSPDLATVSLAFRLLRQGGIKISADVFEKFYDDEGRFKSSLINDVQGLLSLYEAAYMAVRGESILDEAIAFTTTHLKSLVAQDALTPKLAEQINHALARPERKTLPLLEARYFRSFIQSTSDHLYNKTLLNFAKLDFNILLELHKEELNELTKWWKELDFTTKLPYARDRLVALYFFDLGMEFEPQYAFGRKIVTRLNYILSIIDDYYFFYGTLEELELFTEAVQRWNSEAIDTLPEDMKLIYRTLLDAFNEIEEDMAKQGRSHLVRYAKEAFQKVVGAYFVLAKWASEGYVPTIEEYMPIALTSCAMTFVITVSFLGMGDFATKEVFEWISDNPKVVKAASVIGLLLDDMQGHEFEQKIGHVASAIECYTKQHGVSKEEAIKAFEEEVANARKDINEELMKKPQVVARPLLGTILNLARAITFIYKEDDGYTHSYLIKDQIASVLGDELPF

SEQ ID NO: 156 - DNA, 1647 bp, synthetic construct
  source 1..1647: mol_type = other DNA
atgagatctaaagaaactttccgtcctaccgctgacttcaagccatctttgtggagaaaccatttcttgaagggtgcttccgatttcaagaccgttgaccacactgctactcaagaacgtcacgaagctttgaaggaagaagttagaaggatgattactgatgctgaagacaagccagttcaaggtttgagattgatcgatgaagtccaacgtttgggtgtcgcttaccacttcgaaaaggaaatcgaagacgctattcaaaagttgtctccaaactatattcactccaactccccagacttggccaccgtctcattggctttcagactattaagacaaggtggtatcaagatttctgctgatgttttcgaaaagttctacgacgatgaaggtagattcaagtcttctctaattaacgatgtccaaggtttattgtctttgtacgaagctgcttatatggctgtcagaggtgaatccatcttggacgaggctattgctttcaccaccactcatctaaagtccttggtcgctcaagatgctttgactccaaagttagctgagcagatcaaccatgctttggccagaccagaaagaaaaaccttgccattgttggaagcccgttatttcagatccttcatccaatcaacctctgaccatttgtacaacaagaccctgttgaactttgccaagttggatttcaacattttattagaattgcacaaggaagaactgaatgaattgactaagtggtggaaggaattggacttcactactaagttgccatacgctagagacagattggttgccttatacttctttgatttgggtatggaatttgaaccacaatacgccttcggtagaaagatcgttaccagactgaactacatcctctctatcattgatgactactacttcttctacggtaccttggaagaattggaattgttcactgaagctgttcaaagatggaacagtgaagcaattgacaccttgccagaagacatgaaattaatctacagaactttacttgacgctttcaacgaaattgaagaagatatggctaagcaaggtcgttctcacttggtcagatacgctaaagaggctttccaaaaggtcgttggtgcttacttcgtcttggcaaaatgggcttccgaaggttacgttccaactatcgaagaatacatgccaatcgccttgacatcttgtgctatgaccttcgtcattactgtctctttcttgggtatgggtgactttgctaccaaggaagtcttcgaatggattagcgacaacccaaaggttgtcaaggctgcctctgttatcggtttgttgttggacgacatgcaaggtcacgaattcgaacaaaagattggtcacgttgcctccgccatagaatgttacaccaagcaacacggtgtttccaaggaagaagctatcaaggcctttgaagaagaagttgctaacgctagaaaggatatcaacgaagaattgatgaaaaagcctcaagttgttgctagaccattgcttggtactattttgaatttggctagagctatcacttttatctacaaggaagatgatggttacactcactcttacttgatcaaggatcaaattgcttctgttttgggcgacgaattgccattctga

SEQ ID NO: 157 - DNA, 50 bp, synthetic construct
  source 1..50: mol_type = other DNA
catgatatcgacaaaggaaaaggggcctgttcagaatggcaattcgtcgc

SEQ ID NO: 158 - DNA, 52 bp, synthetic construct
  source 1..52: mol_type = other DNA
gtaagaatttttgaaaattcaatataaatgagatctaaagaaactttccgtc

SEQ ID NO: 159 - protein, 548 aa, Citrus maxima
MRSKETFRPTADFKPSLWRNHFLKGASDFKTVDHTATQERHEALKEEVRRMITDAEDKPVQGLRLIDEVQRLGVAYHFEKEIEDAIQKLSPNYIHSNSPDLATVSLAFRLLRQGGIKISADVFEKFYDDEGRFKSSLINDVQGLLSLYEAAYMAVRGESILDEAIAFTTTHLKSLVAQDALTPKLAEQINHALARPLRKTLPRLEARYFRSMIQSTSDHLYNKTLLNFAKLDFNILLELHKEELNELTKWWKELDFTTKLPYARDRLVALYFFDLGMEFEPQYAFGRKIMTQLNYILSIIDDYYFFYGTLEELELFTEAVQRWNIEAVDTLPEYMKLIYRTLLDAFNEIEEDMAKQGRSHLVRYAKEAFQKVVGAYFVLAKWASEGYVPTIEEYMPIALTSCAMTFVITVSFLGMGDFATKEVFEWISDNPKVVKAASVIGLLLDDMQGHEFEQKRGHVASAIECYTKQHGVSKEEAIKAFEEEVANARKDINEELMMKPQVVARPLLGTILNLARAITFIYKEDDGYTHSYLIKDQIASVLGDEVPF

SEQ ID NO: 160 - DNA, 1647 bp, synthetic construct
  source 1..1647: mol_type = other DNA
atgagatctaaggaaactttcagaccaactgctgatttcaagccatctttgtggagaaaccacttcttgaagggtgccagtgatttcaagactgttgaccacactgctacccaagaaagacacgaagctttgaaggaagaagtcagaagaatgattactgatgctgaagacaagccagttcaaggtttgagattaatcgacgaagttcaaagattgggtgttgcctatcatttcgaaaaggaaattgaagacgccattcaaaaattatccccaaactacatccactccaactctccagacttggccaccgttagcttggctttccggttattaagacaaggtggtatcaagatctctgctgacgtcttcgaaaagttctacgacgatgaaggtcgtttcaagtcctcattgattaacgatgtccaaggtttgttgtctttgtacgaagctgcttacatggctgttagaggtgaatctattttggatgaagccattgctttcaccaccactcacttgaagtctctagtggctcaagatgcattgaccccaaagttggctgaacaaatcaaccatgctttggccagaccattgcgtaagaccttgccaagattggaagctcgttatttcagatccatgatccaatctacttccgaccacttatacaacaagacactattgaacttcgctaagttggacttcaatattttgctagaattgcacaaggaagaattgaatgaactcaccaaatggtggaaggaattggactttaccaccaagctaccatacgctagagacagattggttgctttgtacttcttcgatttgggcatggaattcgagccacaatacgccttcggtagaaagatcatgactcaattgaactacattttgtccatcatcgatgactactacttcttttacggtactttggaagaattggaattgttcactgaagctgtccaaagatggaacatcgaagctgtcgacactttgccagaatatatgaaattgatttacagaactttattggatgctttcaacgaaatcgaagaagatatggccaaacaaggtcgttcccatttggtcagatacgctaaggaagctttccaaaaggtcgttggtgcttacttcgtcttggccaagtgggcttctgaaggttacgttccaaccattgaagaatacatgccaatcgctctaacctcttgtgctatgaccttcgttatcactgtctctttcttaggtatgggtgattttgctactaaagaagttttcgaatggatttctgacaacccaaaggttgttaaggccgcttctgtcattggtttgttgttggatgacatgcaaggtcacgaatttgaacaaaagagaggtcacgttgcctccgctattgaatgttacaccaagcaacacggtgtctccaaggaagaagctattaaagcttttgaagaagaagttgctaacgctcgtaaagacatcaacgaagaattgatgatgaagcctcaagttgtcgccagacctctgttgggtaccatcttgaacttggctagagctatcactttcatctacaaggaagatgacggttacacccactcttacttgatcaaggaccaaatagcttctgttttgggtgacgaagtcccattctga

SEQ ID NO: 161 - DNA, 51 bp, synthetic construct
  source 1..51: mol_type = other DNA
catgatatcgacaaaggaaaaggggcctgttcagaatgggacttcgtcacc

SEQ ID NO: 162 - DNA, 52 bp, synthetic construct
  source 1..52: mol_type = other DNA
gtaagaatttttgaaaattcaatataaatgagatctaaggaaactttcagac

SEQ ID NO: 163 - protein, 548 aa, Citrus maxima
MRSKETFRPTADFHPSLWRNHFLKGASDFKTVDHTATQERHEALKEEVRRMITDAEDKPVQKLRLIDEVQRLGVAYHFEKEIEDAIQKLSPNYIHSNSPDLATVSLAFRLLRQGGIKISADVFEKFYDDEGRFKSSLINDVQGLLSLYEAAYMAVRGEHILDEAIAFTTTHLKSLVAQDAVTPKLAEQINHALYRPLRKTLPRLEARYFRSMIQSTSDHLYNKTLLNFAKLDFNILLELHKEELNELTKWWKELDFTTKLPYARDRLVALYFWDLGMEFEPQYAFGRKIMTQLNYILSIIDDTYFFYGTLEELSLFTEAVQRWNIEAVDTLPEYMKLIYRTLLDAFNEIEEDMAKQGRSHLVRYAKEAFQKVVGAYFVLAKWASEGYVPTIEEYMPIALTSCAMTFVITVSFLGMGDFATKEVFEWISDNPKVVKAASVICLLLDDMQGHEFEQKRGHVASAIECYTKQHGVSKEEAIKMFEEEVANARKDINEELMMKPQVVARPLLGTILNLARAIDFIYKEDDGYTHSYLIKDQIASVLGDEVPF

SEQ ID NO: 164 - DNA, 1647 bp, synthetic construct
  source 1..1647: mol_type = other DNA
atgagatcaaaggaaactttccgtccaaccgctgacttccacccatctttgtggagaaaccatttcttgaaaggtgcatctgatttcaagactgttgaccacactgctactcaagaaagacacgaagctttaaaggaagaagtcagaagaatgatcactgacgctgaagacaagccagttcaaaagttgagattgatcgatgaagtccaaagattaggtgttgcctaccacttcgaaaaggaaatcgaagatgctatccagaaattgtctccaaactatattcacagcaactctccagacttggccaccgtctccttggctttcagactgttgagacaaggtggtatcaagatttctgctgatgtcttcgaaaagttctacgatgacgaaggtagattcaagtcttctttgatcaacgatgttcaaggtttgctctctttgtacgaagctgcctatatggctgttcgtggtgaacacattctagatgaagccattgctttcaccacaacccatttgaagtccctcgttgctcaagatgctgtcactccaaagttggctgaacaaatcaaccacgctttataccgtcctcttagaaagaccttacctagattagaagcgcgttatttcagatccatgattcaatctacctccgatcatctctacaacaagaccttgttgaacttcgctaagttggacttcaacattttgttggaattgcacaaggaagagttgaacgaattgactaaatggtggaaggaacttgacttcaccaccaagctgccatacgccagagacagattggtcgccctttacttctgggacttgggtatggaattcgaaccacaatacgctttcggtagaaagatcatgacccaattgaactacatcctaagtatcatcgatgacacttacttcttctacggtactttggaagagttatccttgttcactgaagccgtccaaagatggaacatcgaagctgttgatacgttgccagaatacatgaaattgatttacagaactttgttggacgctttcaacgaaattgaagaagacatggccaagcaaggtagatctcacttggttagatacgctaaggaagccttccaaaaggttgttggtgcttactttgtcttggccaagtgggcatctgaaggttacgttccaactattgaagaatacatgccaatcgctttgacttcttgtgctatgacctttgttattactgtctctttcttgggtatgggtgactttgctaccaaggaagtttttgaatggatctctgacaacccaaaggtcgtcaaggctgcttccgtgatctgtttgctattagatgatatgcaaggtcacgaatttgaacaaaagagaggtcatgtcgcttccgccatcgaatgttacaccaagcaacacggtgtctccaaggaagaagctatcaagatgttcgaagaagaagttgctaacgctagaaaggacattaatgaagaattgatgatgaaaccacaagttgttgctcgtccattgttgggcaccattttgaatttagctagagctattgacttcatttacaaggaagatgacggttacactcactcttacttgatcaaggatcaaattgcctccgttttgggtgacgaagtcccattctga

SEQ ID NO: 165 - DNA, 51 bp, synthetic construct; identical to SEQ ID NO: 161
  source 1..51: mol_type = other DNA

SEQ ID NO: 166 - DNA, 50 bp, synthetic construct
  source 1..50: mol_type = other DNA
gtaagaatttttgaaaattcaatataaatgagatcaaaggaaactttccg

SEQ ID NO: 167 - protein, 548 aa, Citrus maxima
MSSKETFRPTADFHPSLWRNHFLKGASDFKTVDHTATQERHEALKEEVRRMITDAEDKPVQKLRLIDEVQRLGVAYHFEKEIEDAIQKLSPNYIHSNSPDLATVSLAFRLLRQGGIKISCDVFEKFKDDEGRFKSSLINDVQGLLSLYEAAYMAVRGEHILDEAIAFTTTHLKSLVAQDAVTPKLAEQINHALYRPLRKTLPRLEARYFMSMINSTSDHLYNKTLLNFAKLDFNILLELHKEELNELTKWWKELDFTTKLPYARDRLVALYFWDLGTEFEPQYAFGRKIMTQLNYILSIIDDTYDAYGTLEELSLFTEAVQRWNIEAVDTLPEYMKLIYRTLLDAFNEIEEDMAKQGRSHLVRYAKEAFQKVIGAYFVLAKWFSEGYVPTIEEYMPIALTSCAMTFVITVSFLGMGDFATKEVFEWISDNPKVVKAASVICLLLDDMQGHEFEQKRGHVASAIECYTKQHGVSKEEAIKMFEEEVANAWKDINEELMMKPQVVARPLLGTILNLARAIDFIYKEDDGYTHSYLIKDQIASVLGDEVPF

SEQ ID NO: 168 - DNA, 1647 bp, synthetic construct
  source 1..1647: mol_type = other DNA
atgtcttccaaggaaaccttcagaccaactgctgatttccacccatctttgtggagaaaccatttcttaaagggtgcttccgatttcaagactgttgaccacactgccacccaagaaagacacgaagctttgaaggaagaagttagaagaatgatcactgatgctgaagacaagcctgttcaaaagttacgtttgattgacgaagtccaaagactaggtgttgcttaccacttcgaaaaggaaattgaagacgctatccaaaaattgagtccaaactacattcactccaactcaccagacttggctactgtttctttggccttcagattattgagacaaggtggtatcaagatctcttgtgatgttttcgaaaagttcaaggatgacgaaggtagattcaaatcttctttgattaacgatgtccaaggcttgctgtccttatacgaagccgcttacatggctgtccgtggtgaacacatcttggacgaagctattgctttcaccaccacccacttgaagtccttagtggctcaagatgccgttactccaaagttggctgaacaaatcaaccacgctttgtacagaccattgagaaagaccttgccaagattggaagctcgttacttcatgtccatgattaactccacttctgaccatttgtacaacaagacactactcaacttcgctaagttggatttcaacatcttgttggaattgcacaaggaagaattgaacgaattgaccaaatggtggaaggaattagacttcaccactaagttgccatacgccagagacagattggtcgcattgtatttctgggatttgggtaccgaatttgagccacaatacgctttcggtcgtaaaatcatgactcaattgaactacattttgtctatcatagacgatacatacgacgcttacggtactttggaagaactttctttgttcactgaagctgttcaaagatggaacattgaagctgtcgacaccctaccagaatacatgaagttaatttacagaactttgctagacgcctttaatgaaatcgaagaagatatggccaagcaaggtagatctcatttggttagatacgccaaagaagccttccagaaggtcatcggtgcctatttcgtcttggctaagtggttctctgaaggttacgttccaaccattgaagaatatatgccaattgctttgacttcctgcgctatgacttttgttatcaccgtatcattcttgggtatgggtgactttgctaccaaggaagtttttgaatggatttccgacaacccaaaggtcgtcaaggctgcctccgttatctgtttgttgttggacgacatgcaaggtcacgaattcgaacaaaagagaggtcatgttgcttctgctattgaatgttacaccaagcaacacggtgtctctaaggaagaagctatcaagatgttcgaagaagaagtcgctaacgcttggaaggacatcaatgaagaattgatgatgaaacctcaagttgttgctagaccattgttaggtaccattttgaacttggccagagctattgatttcatctacaaggaagatgatggttacactcactcttacttgatcaaggaccaaatcgcgtctgttttgggtgatgaagtcccattttga

SEQ ID NO: 169 - DNA, 52 bp, synthetic construct
  source 1..52: mol_type = other DNA
catgatatcgacaaaggaaaaggggcctgttcaaaatgggacttcatcaccc

SEQ ID NO: 170 - DNA, 48 bp, synthetic construct
  source 1..48: mol_type = other DNA
gtaagaatttttgaaaattcaatataaatgtcttccaaggaaaccttc

SEQ ID NO: 171 - protein, 548 aa, Citrus maxima
MSSKETFRPTADFHPSLWRNHFLKGASDFKTVDHTATQERHEALKEEVRRMITDAEDKPVQKLRLIDEVQRLGVAYHFEKEIEDAIQKLCPNYIHSNSPDLHTVSLAFRLLRQGGIKISCDVFEKFKDDEGRFKSSLINDVQGLLSLYEAAYMAVRGEHILDEAIAFTTTHLKSLVAQDHVTPKLAEQINHALYRPLRKTLPRLEARYFMSMINSTSDHLYNKTLLNFAKLDFNILLELHKEELNELTKWWKELDFTTKLPYARDRLVELYFWDLGTYFEPQYAFGRKIMTQLNYILSIIDDTYDAYGTLEELSLFTEAVQRWNIEAVDTLPEYMKLIYRTLLDAFNEIEEDMAKQGRSHCVRYAKEAFQKVIGAYFVQAKWFSEGYVPTIEEYMPIALTSCAYTFVITNSFLGMGDFATKEVFEWISDNPKVVKAASVICLLLDDMQGHEFEQKRGHVASAIECYTKQHGVSKEEAIKMFEEEVANAWKDINEELMMKPTVVARPLLGTILNLARAIDFIYKEDDGYTHSYLIKDQIASVLGDHVPF

SEQ ID NO: 172 - DNA, 1647 bp, synthetic construct
  source 1..1647: mol_type = other DNA
atgtcttccaaggaaactttcagaccaactgctgacttccacccatctttgtggagaaatcatttcttgaagggtgcttctgacttcaaaactgtcgatcacaccgccacccaagaaagacacgaagctttgaaagaagaagtcagaagaatgatcactgatgctgaagacaagcctgtccaaaaattgagattgattgatgaagtccaaagactaggtgttgcttaccacttcgaaaaggaaatcgaggatgctatccaaaagttgtgtccaaactacattcactccaactctccagatttgcacactgtttccttggctttcagattattgagacaaggtggtattaagatttcatgtgatgtctttgaaaagttcaaggatgatgaaggtagattcaagtcttctttgatcaacgatgtccaaggtttgttgtccctatacgaagccgcttatatggctgtcagaggtgaacacattttggacgaagctattgctttcactaccactcacttgaagagcctagtcgctcaagatcatgtcactccaaagttggctgaacaaatcaaccacgctttgtacagacctcttagaaagaccttaccaagattggaagctcgttatttcatgtccatgattaattctacctccgaccatttgtacaacaagactctcttgaacttcgctaagttggatttcaacattttgttggaattgcacaaggaagaattaaacgaattgaccaaatggtggaaagaactagatttcaccaccaagttgccatacgctagagacagattggttgaattatacttctgggacttgggcacctactttgaaccacaatacgccttcggtcggaagatcatgactcaattgaactatatcttgtccatcatcgatgacacttacgacgcttacggtactctggaagaattgtctttattcactgaagctgtccaaagatggaacatcgaagctgttgacaccttgccagaatacatgaaattaatttaccgtactttgttggacgcatttaatgaaattgaagaagacatggccaagcaaggtcgtagtcattgcgttagatacgctaaggaagctttccaaaaggttattggtgcttacttcgttcaggctaagtggttctctgaaggttacgttccaaccattgaagaatacatgccaatcgccttgacttcttgtgcttacacctttgtgatcaccaactctttcttgggtatgggtgactttgctaccaaggaagttttcgaatggatttccgacaacccaaaggtcgtcaaggctgcctccgttatctgtttgttattggacgacatgcaaggtcacgaattcgaacaaaagagaggtcacgttgcctctgctatcgaatgttacactaaacaacacggtgtctctaaggaagaagccatcaagatgttcgaagaagaagttgctaacgcttggaaggacatcaacgaagaattgatgatgaagccaacagttgttgccagaccattgttaggtactatcttgaacttggcgcgtgccattgacttcatctacaaggaagatgacggttacacccactcttacttgattaaggaccaaatagcttctgttttgggtgatcatgttccattctga

SEQ ID NO: 173 - DNA, 54 bp, synthetic construct
  source 1..54: mol_type = other DNA
gatatcgacaaaggaaaaggggcctgttcagaatggaacatgatcacccaaaac

SEQ ID NO: 174 - DNA, 50 bp, synthetic construct
  source 1..50: mol_type = other DNA
gtaagaatttttgaaaattcaatataaatgtcttccaaggaaactttcag

SEQ ID NO: 175 - DNA, 54 bp, synthetic construct
  source 1..54: mol_type = other DNA
tactttaacgtcaaggagaaaaaactataatgtcttctggtgaaactttcagac

SEQ ID NO: 176 - DNA, 44 bp, synthetic construct
  source 1..44: mol_type = other DNA
ctatcgatttcaattcaattcaattcagaatgggacgtggtcac

SEQ ID NO: 177 - DNA, 59 bp, synthetic construct
  source 1..59: mol_type = other DNA
aaaggtctcagatctgagtccatcctacaaagtcgttttagagctagaaatagcaagtt

SEQ ID NO: 178 - DNA, 42 bp, synthetic construct
  source 1..42: mol_type = other DNA
aaaggtctcaaaactctagactttttcgatgatgtagtttct